European Patent Specification EP 4 039 710 B1, published March 25, 2026. Title: Anti-CD3 antibodies, anti-CD123 antibodies and bispecific antibodies specifically binding to CD3 and/or CD123. Applicant: SANOFI. The sequence listing filed with the application follows.

SEQUENCE LISTING (400 sequences)

SEQ ID NO: 1 - protein, 207 aa, Homo sapiens
MQSGTHWRVLGLCLLSVGVWGQDGNEEMGGITQTPYKVSISGTTVILTCPQYPGSEILWQHNDKNIGGDEDDKNIGSDEDHLSLKEFSELEQSGYYVCYPRGSKPEDANFYLYLRARVCENCMEMDVMSVATIVIVDICITGGLLLLVYYWSKNRKAKAKPVTRGAGAGGRQRGQNKERPPPVPNPDYEPIRKGQRDLYSGLNQRRI

SEQ ID NO: 2 - protein, 198 aa, Macaca fascicularis
MQSGTRWRVLGLCLLSIGVWGQDGNEEMGSITQTPYQVSISGTTVILTCSQHLGSEAQWQHNGKNKEDSGDRLFLPEFSEMEQSGYYVCYPRGSNPEDASHHLYLKARVCENCMEMDVMAVATIVIVDICITLGLLLLVYYWSKNRKAKAKPVTRGAGAGGRQRGQNKERPPPVPNPDYEPIRKGQQDLYSGLNQRRI

SEQ ID NO: 3 - protein, 340 aa, Homo sapiens
  DOMAIN (1)..(104): extracellular domain of human CD3 epsilon
  MISC_FEATURE (105)..(340): His-tagged FC-Fusion
DGNEEMGGITQTPYKVSISGTTVILTCPQYPGSEILWQHNDKNIGGDEDDKNIGSDEDHLSLKEFSELEQSGYYVCYPRGSKPEDANFYLYLRARVCENCMEMDGSDKTHTCPPCPAPELLGGPSVFLFPPKPKDTLMISRTPEVTCVVVDVSHEDPEVKFNWYVDGVEVHNAKTKPREEQYNSTYRVVSVLTVLHQDWLNGKEYKCKVSNKALPAPIEKTISKAKGQPREPQVYTLPPSRDELTKNQVSLTCLVKGFYPSDIAVEWESNGQPENNYKTTPPVLDSDGSFFLYSKLTVDKSRWQQGNVFSCSVMHEALHNHYTQKSLSLSPGHHHHHHHH

SEQ ID NO: 4 - protein, 333 aa, Macaca fascicularis
  Domain (1)..(95): extracellular domain of Macaca fascicularis CD3epsilon protein
  MISC_FEATURE (96)..(333): Fc fusion
DGNEEMGSITQTPYQVSISGTTVILTCSQHLGSEVQWQHNGKNKEDSGDRLFLPEFSEMEQSGYYVCYPRGSNPEDASHHLYLKARVCENCMEMDGSDKTHTCPPCPAPELLGGPSVFLFPPKPKDTLMISRTPEVTCVVVDVSHEDPEVKFNWYVDGVEVHNAKTKPREEQYNSTYRVVSVLTVLHQDWLNGKEYKCKVSNKALPAPIEKTISKAKGQPREPQVYTLPPSRDELTKNQVSLTCLVKGFYPSDIAVEWESNGQPENNYKTTPPVLDSDGSFFLYSKLTVDKSRWQQGNVFSCSVMHEALHNHYTQKSLSLSPGSAWSHPQFEK

SEQ ID NO: 5 - protein, 121 aa, Artificial Sequence
  VH of the so-called "20G6-F3" anti-CD3 antibody
EVQLVETGGSLVQPGKSLKLTCATSGFTFTKAWMHWVRQSPEKQLEWVAQIKDKSNSYATYYAESVKGRFTISRDDSKSTIYLQMNSLKEEDTAIYYCRGVYYALSPFDYWGQGVMVTVSS

SEQ ID NO: 6 - protein, 8 aa, Artificial Sequence
  CDR1-H of the so-called "20G6-F3" anti-CD3antibody
GFTFTKAW

SEQ ID NO: 7 - protein, 10 aa, Artificial Sequence
  CDR2-H of the so-called "20G6-F3" anti-CD3antibody
IKDKSNSYAT

SEQ ID NO: 8 - protein, 12 aa, Artificial Sequence
  CDR3-H of the so-called "20G6-F3" anti-CD3antibody
RGVYYALSPFDY

SEQ ID NO: 9 - protein, 112 aa, Artificial Sequence
  VL of the so-called "20G6-F3" anti-CD3 antibody
DVVMTQTPVSLSVSLGGQVSISCRSSQSLVHNNGNTYLSWYLQKPGQSPQSLIYKVSNRFSGFSDRFSGSGSGTDFTLKISRVDPDDLGVYYCGQGTQYPFTFGSGTKLEIK

SEQ ID NO: 10 - protein, 11 aa, Artificial Sequence
  CDR1-L of the so-called called "20G6-F3", "11D7-C3" , "13H2-C2" , "13C1-F6", "1E6-C9, "10F4-C10", "18G9-H11", "12G3-E8", "5B1-G2", "16F8-A7", "11F9-F8", "8C2-F7", "20E5-F10" and "3H6-D2" anti-CD3 antibodies
QSLVHNNGNTY

SEQ ID NO: 11 - protein, 9 aa, Artificial Sequence
  CDR3-L of the so-called "20G6-F3", "4B4-D7" , "11H3-E5"  , "13H2-C2", "13C1-F6", "10F4-C10", "4E7-C9", "11F3-B9", "12G3-E8", "5B1-G2", "6F4-D10", "16F8-A7", "20E5-F10" and "3H6-D2" anti-CD3 antibodies
GQGTQYPFT

SEQ ID NO: 12 - protein, 121 aa, Artificial Sequence
  VH of the so-called "4B4-D7" anti-CD3 antibody.
EVQLVETGGRLVQPGRSLKLTCATSGFTFSNAWMHWVRQSPEKQLEWVAQIKARSNNYATYYAESVKGRFTISRDDSKSTIYLQMNSLKEEDTAIYYCRGTYYASKPFDYWGQGVMVTVSS

SEQ ID NO: 13 - protein, 8 aa, Artificial Sequence
  CDR3-L of the so-called "20G6-F3", "4B4-D7" , "11H3-E5"  , "13H2-C2", "13C1-F6", "10F4-C10", "4E7-C9", "11F3-B9", "12G3-E8", "5B1-G2", "16F8-A7", "20E5-F10" and "3H6-D2" anti-CD3 antibodies.
GFTFSNAW

SEQ ID NO: 14 - protein, 10 aa, Artificial Sequence
  CDR2-H of the so-called "4B4-D7" anti-CD3 antibody
IKARSNNYAT

SEQ ID NO: 15 - protein, 12 aa, Artificial Sequence
  CDR3-H of the so-called "4B4-D7" anti-CD3 antibody.
RGTYYASKPFDY

SEQ ID NO: 16 - protein, 112 aa, Artificial Sequence
  VL of the so-called "4B4-D7" anti-CD3 antibody
DVVMTQTPVSLSVSLGGQVSISCRSSQSLVHDNGNTYLSWSLQRPGQSPQVLIYKVSNRFSGTSDRFTGSGSGTDFTLKISRVEPDDLGVYYCGQGTQYPFTFGSGTKLEIK

SEQ ID NO: 17 - protein, 11 aa, Artificial Sequence
  CDR1-L of the so-called "4B4-D7", "11H3-E5" and "11F3-B9" anti-CD3 antibodies.
QSLVHDNGNTY

SEQ ID NO: 18 - protein, 122 aa, Artificial Sequence
  VH of the so-called "4E7-C9" anti-CD3 antibody
EVQVVETGGSLVQPGKSLKLTCATSGFTFSNAWMHWVRQSPEKQLEWVAQIKDKSNNYATYYAESLKGRFTISRDDPKRSIYLQMNSLREEDTAIYYCRYVHYGIGYAMDAWGQGTSVTVSS

SEQ ID NO: 19 - protein, 10 aa, Artificial Sequence
  CDR2-H of the so-called "4E7-C9", "18F5-H10", "20E5-F10" and "3H6-D2" anti-CD3 antibodies
IKDKSNNYAT

SEQ ID NO: 20 - protein, 13 aa, Artificial Sequence
  CDR3-H of the so-called "4E7-C9" anti-CD3 antibody
RYVHYGIGYAMDA

SEQ ID NO: 21 - protein, 112 aa, Artificial Sequence
  VL of the so-called "4E7-C9" anti-CD3 antibody
DVVMTQTPVSLSVSLGGQVSISCRSSQSLEHNNGNTYLSWYLQKPGQSPQPLIYKVSNRFSGISDRFSGSGSGTDFTLKISRVEPDDLGVYYCGQGTQYPFTFGPGTKLELK

SEQ ID NO: 22 - protein, 11 aa, Artificial Sequence
  CDR1-H of the so-called "4E7-C9" anti-CD3 antibody
QSLEHNNGNTY

SEQ ID NO: 23 - protein, 122 aa, Artificial Sequence
  VH of the so-called "18F5-H10" anti-CD3 antibody
EVQVVETGGSLVQPGKSLKLTCATSGFTFTNAWMHWVRRSPEKQLEWVAQIKDKSNNYATYYAESVKGRFTISRDDSKSSIYLQMNSLKEEDTAIYYCRYVHYRFAYALDAWGRGTSVSVSS

SEQ ID NO: 24 - protein, 8 aa, Artificial Sequence
  CDR1-H of the so-called "18F5-H10" anti-CD3 antibody
GFTFTNAW

SEQ ID NO: 25 - protein, 13 aa, Artificial Sequence
  CDR3-H of the so-called "18F5-H10" anti-CD3 antibody
RYVHYRFAYALDA

SEQ ID NO: 26 - protein, 112 aa, Artificial Sequence
  VL of the so-called "18F5-H10" anti-CD3 antibody
DVLMTQTPVSLSVSLGGQVSISCRSSQSLVHTNGNTYLSWYLQKPGQSPQLLIYKVSNRLSGISDRFSGSGSGTDFTLKISRVEPDDLGVYYCGQGTHYPFTFGAGTKLELK

SEQ ID NO: 27 - protein, 11 aa, Artificial Sequence
  CDR1-L of the so-called "18F5-H10" anti-CD3 antibody
QSLVHTNGNTY

SEQ ID NO: 28 - protein, 9 aa, Artificial Sequence
  CDR3-L of the so-called "18F5-H10", "11D7-C3", "1E6-C9" and "10E6-G6" anti-CD3 antibodies
GQGTHYPFT

SEQ ID NO: 29 - protein, 118 aa, Artificial Sequence
  VH of the so-called "12D2-E5" anti-CD3 antibody
EVKLVESGGGLVQPGRSLRLSCAASGFNFYAYWMGWVRQAPGKGLEWIGEIKKDGTTINYTPSLKDRFTISRDNAQNTLYLQMTKLGSEDTALYYCAREERDGYFDYWGQGVMVTVSS

SEQ ID NO: 30 - protein, 8 aa, Artificial Sequence
  CDR1-H of the so-called "12D2-E5" anti-CD3 antibody
GFNFYAYW

SEQ ID NO: 31 - protein, 8 aa, Artificial Sequence
  CDR2-H of the so-called "12D2-E5" anti-CD3 antibody
IKKDGTTI

SEQ ID NO: 32 - protein, 11 aa, Artificial Sequence
  CDR3-H of the so-called "12D2-E5" and "3G5-E10" anti-CD3 antibody
AREERDGYFDY

SEQ ID NO: 33 - protein, 109 aa, Artificial Sequence
  VL of the so-called "12D2-E5" anti-CD3 antibody.
QFVLTQPNSVSTNLGSTVKLSCKRSTGNIGSNYVNWYQQHEGRSPTTMIYRDDKRPDGVPDRFSGSIDRSSNSALLTINNVQTEDEADYFCQSYSSGIVFGGGTKLTVL

SEQ ID NO: 34 - protein, 8 aa, Artificial Sequence
  CDR1-H of the so-called "12D2-E5" anti-CD3 antibody
TGNIGSNY

SEQ ID NO: 35 - protein, 8 aa, Artificial Sequence
  CDR3-H of the so-called "12D2-E5" anti-CD3 antibody
QSYSSGIV

SEQ ID NO: 36 - protein, 121 aa, Artificial Sequence
  VH of the so-called "11D7-C3" anti-CD3 antibody
EVQFVETGGSLVQPGKSLKLTCATSGFTFSNAWMHWVRQSPEKQLEWVAQIKAKSNNYATYYAESVKGRFTISRDDSKSSVYLQMNSLKEEDTATYYCRGLYYGLSPSDYWGQGVMVTVSS

SEQ ID NO: 37 - protein, 10 aa, Artificial Sequence
  CDR2-H of the so-called "11D7-C3", "11H3-E5", "13H2-C2", "13C1-F6", "1E6-C9", "10F4-C10", "18G9-H11", "11F3-B9", "6F4-D10", "16F8-A7", "11F9-F8" and "20B5-F10" anti-CD3 antibodies
IKAKSNNYAT

SEQ ID NO: 38 - protein, 12 aa, Artificial Sequence
  CDR3-H of the so-called "11D7-C3" anti-CD3 antibody
RGLYYGLSPSDY

SEQ ID NO: 39 - protein, 112 aa, Artificial Sequence
  VL of the so-called "11D7-C3" anti-CD3 antibody.
DVVMTQTPVSLSVSLGGQVSISCRSSQSLVHNNGNTYLSWYLQKPGQSPQLLIYKVSNRFSGISDRFSGSGSGTDFTLKISRVEPDDLGVYYCGQGTHYPFTFGSGTKLEIK

SEQ ID NO: 40 - protein, 121 aa, Artificial Sequence
  VH of the so-called "11H3-E5" anti-CD3 antibody
EVQLVETGGSLVQPGKSLKLTCATSGFTFSNAWMHWVRQSPEKQLEWVAQIKAKSNNYATYYAESVKGRFTISRDDSKSSVYLQMNSLKEEDTAIYYCRGTYYAYKPFDYWGQGVMVTVSS

SEQ ID NO: 41 - protein, 12 aa, Artificial Sequence
  CDR3-H of the so-called called "11H3-E5" anti-CD3 antibody
RGTYYAYKPFDY

SEQ ID NO: 42 - protein, 112 aa, Artificial Sequence
  VL of the so-called "11H3-E5" anti-CD3 antibody
DVVMTQTPVSLSVSLGGQVSISCRSSQSLVHDNGNTYLSWSLQKPGQSPQVLIYKVSNRFSGTSDRFTGSGSGTDFTLKISRVEPDDLGVYYCGQGTQYPFTFGSGTKLEIK

SEQ ID NO: 43 - protein, 121 aa, Artificial Sequence
  VH of the so-called "13H2-C2" anti-CD3 antibody.
EEELVETGGSLVQPGKSLKLTCATSGFTFSNAWMHWVRQSPDKQLEWVAQIKAKSNNYATYYAESVKGRFTISRDDSKSSVYLQMNNLKEEDTAIYYCRYVHYGLAPMDAWGQGTSVTVSS

SEQ ID NO: 44 - protein, 12 aa, Artificial Sequence
  CDR3-H of the so-called "13H2-C2" anti-CD3 antibody
RYVHYGLAPMDA

SEQ ID NO: 45 - protein, 112 aa, Artificial Sequence
  VL of the so-called "13H2-C2" anti-CD3 antibody
DVVMTQTPVSLSVSLGGQVSISCRSSQSLVHNNGNTYLSWYLQKAGQSPQLLIYKVSNRFSGISDRFSGSGSGTDFILKISRVEPDDLGVFYCGQGTQYPFTFGAGTKLELK

SEQ ID NO: 46 - protein, 121 aa, Artificial Sequence
  VH of the so-called "13C1-F6" and "11F9-F8" anti-CD3 antibodies
EVQLVETGGTLVQPGKSLKLTCATSGFTFSNAWMHWVRQSPEKQLEWVAQIKAKSNNYATYYAESVKGRFTISRDDSKTSVYLQLNSLREEDTAIYYCRGTQYGYNPFDYWGQGVMVTVSS

SEQ ID NO: 47 - protein, 12 aa, Artificial Sequence
  CDR3-H of so-called "13C1-F6", "10E6-G6" and "11F9-F8" anti-CD3 antibodies
RGTQYGYNPFDY

SEQ ID NO: 48 - protein, 112 aa, Artificial Sequence
  VL of the so-called "13H2-C2" anti-CD3 antibody
DVVMTQSPVSLSVSLGGQVSISCRSSQSLVHNNGNTYLSWYLQRSGQSPQLLIYKVSNRLSGISDRFSGSGSGTDFTLKISRIEPDDLGVYYCGQGTQYPFTFGSGTRLEIK

SEQ ID NO: 49 - protein, 118 aa, Artificial Sequence
  VH of the so-called "18H11-F10" anti-CD3 antibody
EVQLVESGGGLVQPGRSLKLSCAASGFIFSDYYMAWVRQAPKKGLEWVATISISGSRTYYPDSVKGRFTVSRDNAKSSLYLQMNSLKSEDTATYYCATNNPGGWFVYWGQGTLVTVSS

SEQ ID NO: 50 - protein, 8 aa, Artificial Sequence
  CDR1-H of the so-called  "18H11-F10" anti-CD3 antibody
GFIFSDYY

SEQ ID NO: 51 - protein, 8 aa, Artificial Sequence
  CDR2-H of the so-called  "18H11-F10" anti-CD3 antibody
ISISGSRT

SEQ ID NO: 52 - protein, 11 aa, Artificial Sequence
  CDR3-H of the so-called  "18H11-F10" anti-CD3 antibody
ATNNPGGWFVY

SEQ ID NO: 53 - protein, 106 aa, Artificial Sequence
  VL of the so-called "18H11-F10" anti-CD3 antibody
NIQMTQSPSLLSASVGDRVTLSCKAGQNINNDLAWYQQKLGEAPRLLIYNANSLQTGIPSRFSGSGSGADFTLTISSLQPEDVATYFCQQYSSGDTFGAGTKLELK

SEQ ID NO: 54 - protein, 6 aa, Artificial Sequence
  CDR1-L of the so-called  "18H11-F10" anti-CD3 antibody
QNINND

SEQ ID NO: 55 - protein, 8 aa, Artificial Sequence
  CDR3-L of the so-called "18H11-F10" anti-CD3 antibody
QQYSSGDT

SEQ ID NO: 56 - protein, 121 aa, Artificial Sequence
  VH of the so-called "1E6-C9" anti-CD3 antibody
EVQLVETGGSLVQPGKSLKLTCATSGFTFSYAWMHWVRQSPDKQLQWVAQIKAKSNNYATYYAESVEGRFTISRDDSKSSVYLQMNSLKEEDTAIYYCRGVYYGLLGLDAWGQGTSVTVSS

SEQ ID NO: 57 - protein, 8 aa, Artificial Sequence
  CDR1-H of the so-called "1E6-C9" anti-CD3 antibody
GFTFSYAW

SEQ ID NO: 58 - protein, 12 aa, Artificial Sequence
  CDR3-H of the so-called "1E6-C9" anti-CD3 antibody
RGVYYGLLGLDA

SEQ ID NO: 59 - protein, 112 aa, Artificial Sequence
  VL of the so-called "1E6-C9" anti-CD3 antibody
DVVMTQTPVSLSVRLGGQVSISCRSSQSLVHNNGNTYLSWFLQKPGQSPQLLIYKVSNRFSGISDRFSGSASGTDFTLKISRVEPDDLGVYYCGQGTHYPFTFGSGTKLEIK

SEQ ID NO: 60 - protein, 121 aa, Artificial Sequence
  VH of the so-called "10F4-C10" anti-CD3 antibody
EVQLVETGGSLVQPGKSLKITCATSGFTFSNAWMHWVRQSPEKQLEWVAQIKAKSNNYATYYAESVKGRFTISRDDSKSSIYLQMNSLKEEDTAIYYCRAVNYGNYPLDYWGQGVMVTVSS

SEQ ID NO: 61 - protein, 12 aa, Artificial Sequence
  CDR3-H of the so-called "10F4-C10" anti-CD3 antibody
RAVNYGNYPLDY

SEQ ID NO: 62 - protein, 112 aa, Artificial Sequence
  VL of the so-called "10F4-C10" anti-CD3 antibody
DVVMTQTPVSLSVSLGGQVSISCRSSQSLVHNNGNTYLSWCLQKPGQSPQLLIYKVSNRFSGISDRFSGSGSGTDFTLKISRVEPDDLGVYYCGQGTQYPFTFGAGTKLELK

SEQ ID NO: 63 - protein, 121 aa, Artificial Sequence
  VH of the so-called "10E6-G6" anti-CD3 antibody
EVQLVETGGGLVQSGKSLKLTCATSGFTVTNAWMHWVRQSPEKQLEWVAQIKAKSNNYETYYAESVKGRFTISRDDSKSSVYLQMNSLKEEDTAIYYCRGTQYGYNPFDYWGQGVMVTVSS

SEQ ID NO: 64 - protein, 8 aa, Artificial Sequence
  CDR1-H of the so-called "10E6-G6" anti-CD3 antibody
GFTVTNAW

SEQ ID NO: 65 - protein, 10 aa, Artificial Sequence
  CDR3-H of the so-called "10E6-G6" anti-CD3 antibody
IKAKSNNYET

SEQ ID NO: 66 - protein, 112 aa, Artificial Sequence
  VL of the so-called "10E6-G6" anti-CD3 antibody
DVVMTQSPVSLSVSLGGQVSISCRSSQSLVHNNGYTYLSWYLQKPGQSPQVFIYKVSNRFSGISDRFSGSGSGTDFTLKISRIEPDDLGVYYCGQGTHYPFTFGSGTKLEIK

SEQ ID NO: 67 - protein, 11 aa, Artificial Sequence
  CDR1-L of the so-called "10E6-G6" anti-CD3 antibody
QSLVHNNGYTY

SEQ ID NO: 68 - protein, 122 aa, Artificial Sequence
  VH of the so-called "18G9-H11" anti-CD3 antibody
EVQLVETGGSLVQPGKSLKLTCATSGFTFSNAWIQWVRQSPEKQLEWVAQIKAKSNNYATYYAESVKGRFTISRDDSKSSVYLQMNSLKEEDTALYYCTWRHYYSSHTMDAWGQGTLVTVSS

SEQ ID NO: 69 - protein, 13 aa, Artificial Sequence
  CDR3-H of the so-called "18G9-H11" anti-CD3 antibody
TWRHYYSSHTMDA

SEQ ID NO: 70 - protein, 112 aa, Artificial Sequence
  VL of the so-called "18G9-H11" anti-CD3 antibody
DVVMTQTPVSLSVSLGGQVSISCRSSQSLVHNNGNTYLSWYLQKPGQSPQLLIYKVSNRFSGISDRFSGSGSGTDFTLKISRVAPTDLGVYYCGQGSQYPFTFGAGTKLELK

SEQ ID NO: 71 - protein, 9 aa, Artificial Sequence
  CDR3-L of the so-called "18G9-H11" anti-CD3 antibody
GQGSQYPFT

SEQ ID NO: 72 - protein, 121 aa, Artificial Sequence
  VH of the so-called "11F3-B9" anti-CD3 antibody
EVQLVETGGSLVQPGKSLTLTCATSGFTFSNAWMHWVRQSPEKQLEWVAQIKAKSNNYATYYAESVKGRFTISRDDSKRSVYLQMNSLKEEDTAIYYCRYVNYGLAPMDVWGQGTSVTVSS

SEQ ID NO: 73 - protein, 112 aa, Artificial Sequence
  VL of the so-called "11F3-B9" anti-CD3 antibody
DVVMTQTPVSLSVSLGGQVSISCRSSQSLVHDNGNTYLSWYLQKPGQSPQLLIYKVSNRFSGFSDRFSGSGSGTDFTLKISRVEPDDLGVYYCGQGTQYPFTFGAGTKLELK

SEQ ID NO: 74 - protein, 123 aa, Artificial Sequence
  VH of the so-called "12G3-E8" anti-CD3 antibody
EVRVVETGGSLVQPGKSLKLTCATSGFTFSLAWMHWVRQSPEKKLEWVAQIKDKANNYATYYAESVKGRFTISRDDSKRSVYLQMNRLKEEDTAIYYCRGVYYGFSMTPFDYWGQGVMVTVSS

SEQ ID NO: 75 - protein, 8 aa, Artificial Sequence
  CDR1-H of the so-called "18G9-H11" anti-CD3 antibody
GFTFSLAW

SEQ ID NO: 76 - protein, 10 aa, Artificial Sequence
  CDR2-H of the so-called "18G9-H11" anti-CD3 antibody
IKDKANNYAT

SEQ ID NO: 77 - protein, 14 aa, Artificial Sequence
  CDR3-H of the so-called "18G9-H11" anti-CD3 antibody
RGVYYGFSMTPFDY

SEQ ID NO: 78 - protein, 112 aa, Artificial Sequence
  VL of the so-called "12G3-E8" anti-CD3 antibody
DVAMTQTPVSLSVSLGGQVSISCRSSQSLVHNNGNTYLSWYLQKPGQSPQVLIYKVSNRFSGISDRFSGSGSGADFTLKISRVEPDDLGVYYCGQGTQYPFTFGAGTKLELK

SEQ ID NO: 79 - protein, 121 aa, Artificial Sequence
  VH of the so-called "5B1-G2" anti-CD3 antibody
EVQVVETGGSLVQPGKSLKLTCATSGFSFSNAWMHWVRQSPEKQLEWVAQIKDKANNYATYYAESVKGRFTISRDDSKGSIYLQMNSLKEEDTAVYYCRGLYYGLFPSDYWGQGVMVTVSS

SEQ ID NO: 80 - protein, 8 aa, Artificial Sequence
  CDR1-H of the so-called "5B1-G2" anti-CD3 antibody
GFSFSNAW

SEQ ID NO: 81 - protein, 12 aa, Artificial Sequence
  CDR3-H of the so-called "5B1-G2" anti-CD3 antibody
RGLYYGLFPSDY

SEQ ID NO: 82 - protein, 112 aa, Artificial Sequence
  VL of the so-called "5B1-G2" anti-CD3 antibody
DVVMTQTPVSLSVSLGGQVSISCRSSQSLVHNNGNTYLSWYLLKPGQSPQLLIYKVSNRFSGISDRFSGGGSGTDFTLKISRLEPDDLGIYYCGQGTQYPFTFGSGTKLEIK

SEQ ID NO: 83 - protein, 117 aa, Artificial Sequence
  part of VH of the so-called "16F8-A7" anti-CD3 antibody
VETGGNLVQPGKSLKLTCATSGFTFSNAWMHWVRQSPEKQLEWVAQIKAKSNNYATYYAESVKGRFTISRDDSKSSVYLQMNSLKEEDTAIYYCRYVNYGLAPMDVWGQGTSVTVSS

SEQ ID NO: 84 - protein, 12 aa, Artificial Sequence
  CDR3-H of the so-called "16F8-A7" and "11F3-B9" anti-CD3 antibodies
RYVNYGLAPMDV

SEQ ID NO: 85 - protein, 112 aa, Artificial Sequence
  VL of the so-called "16F8-A7" anti-CD3 antibody
DVVMTQTPVSLSVSLGGQVSISCRSSQSLVHNNGNTYLSWYLQKPGQSPQLLIYKVSNRFSGFSDRFSGSGSGTDFTLKISRVEPDDLGVYYCGQGTQYPFTFGAGTKLELK

SEQ ID NO: 86 - protein, 171 aa, Homo sapiens
MEHSTFLSGLVLATLLSQVSPFKIPIEELEDRVFVNCNTSITWVEGTVGTLLSDITRLDLGKRILDPRGIYRCNGTDIYKDKESTVQVHYRMCQSCVELDPATVAGIIVTDVIATLLLALGVFCFAGHETGRLSGAADTQALLRNDQVYQPLRDRDDAQYSHLGGNWARNK

SEQ ID NO: 87 - protein, 112 aa, Artificial Sequence
  VL of the so-called "11F9-F8" anti-CD3 antibody
DVVLTQTPVSLSVSLGGQVSISCRSSQSLVHNNGNTYLSWSLQKPGQSPQVLIYKVSNRFSGISNRFSGSGSGTDFTLKISRVEPDDLGVYYCGQGAHYPFTFGSGTKLEIK

SEQ ID NO: 88 - protein, 9 aa, Artificial Sequence
  CDR3-L of the so-called "11F9-F8" anti-CD3 antibody
GQGAHYPFT

SEQ ID NO: 89 - protein, 118 aa, Artificial Sequence
  VH of the so-called "3G5-E10" anti-CD3 antibody
EVKLVESGGGLVQPGRSLKLSCAASGFNFNVYWMGWVRQAPGKGLEWIGEIKKDSNSINYTPSLKEKFTISRDNAQNTLYLQVNKLGSEDTAIYYCAREERDGYFDYWGQGVMVTVSS

SEQ ID NO: 90 - protein, 8 aa, Artificial Sequence
  CDR1-H of the so-called "3G5-E10" anti-CD3 antibody
GFNFNVYW

SEQ ID NO: 91 - protein, 8 aa, Artificial Sequence
  CDR2-H of the so-called "3G5-E10" anti-CD3 antibody
IKKDSNSI

SEQ ID NO: 92 - protein, 107 aa, Artificial Sequence
  VL of the so-called "3G5-E10" anti-CD3 antibody
NIVMTQSPKSMSMSVGERVTLTCKASENVVTYVSWYQQKPEQSPKLLIYGASNRYTGVPDRFTGSGSATDFTLTISSVQAEDLADYHCGQGYSYPYTFGGGTKLEIK

SEQ ID NO: 93 - protein, 6 aa, Artificial Sequence
  CDR1-L of the so-called "3G5-E10" anti-CD3 antibody
ENVVTY

SEQ ID NO: 94 - protein, 9 aa, Artificial Sequence
  CDR3-L of the so-called "3G5-E10" anti-CD3 antibody
GQGYSYPYT

SEQ ID NO: 95 - protein, 119 aa, Artificial Sequence
  VH of the so-called "9D7-F3" anti-CD3 antibody
AVQLVESGGGLVQPKESLKISCAASGFTFSNAAMYWVRQAPGKGLEWVARIRTKPNNYATYYADSVTGRFIISRDDSRSMVYLQMDNLQTEDTAMYYCTALISTAMAAWGQGTSVTVSS

SEQ ID NO: 96 - protein, 8 aa, Artificial Sequence
  CDR1-H of the so-called "9D7-F3" anti-CD3 antibody
GFTFSNAA

SEQ ID NO: 97 - protein, 10 aa, Artificial Sequence
  CDR2-H of the so-called "9D7-F3" anti-CD3 antibody
IRTKPNNYAT

SEQ ID NO: 98 - protein, 10 aa, Artificial Sequence
  CDR3-H of the so-called "9D7-F3" anti-CD3 antibody
TALISTAMAA

SEQ ID NO: 99 - protein, 106 aa, Artificial Sequence
  VL of the so-called "9D7-F3" anti-CD3 antibody
DIQMTQSPSFLSASVGDRVTINCKASQNINKYLNWYHQMLGEAPKLVISNTNNLQAGIPSRFSGSGSGTDFTLTISSLQPEDVATYFCLQHRSGYTFGLGTKLELK

SEQ ID NO: 100 - protein, 6 aa, Artificial Sequence
  CDR1-L of the so-called "9D7-F3" and "6C9-C9" anti-CD3 antibody
QNINKY

SEQ ID NO: 101 - protein, 8 aa, Artificial Sequence
  CDR3-L of the so-called "9D7-F3" anti-CD3 antibody
LQHRSGYT

SEQ ID NO: 102 - protein, 114 aa, Artificial Sequence
  VH of the so-called "8C2-F7" anti-CD3 antibody
QIQLVQSGPELKKPGESVKISCKASGYTFTDFAMNWVKQAPGNGLKWMGWINTQTGKPTYADGFKQRFVFSLETSASTIYLQINNLNIEDTATYFCTRGALASVGQGVLVTVSS

SEQ ID NO: 103 - protein, 8 aa, Artificial Sequence
  CDR1-H of the so-called "8C2-F7" anti-CD3 antibody
GYTFTDFA

SEQ ID NO: 104 - protein, 8 aa, Artificial Sequence
  CDR2-H of the so-called "8C2-F7" anti-CD3 antibody
INTQTGKP

SEQ ID NO: 105 - protein, 7 aa, Artificial Sequence
  CDR3-H of the so-called "8C2-F7" anti-CD3 antibody
TRGALAS

SEQ ID NO: 106 - protein, 112 aa, Artificial Sequence
  VL of the so-called "8C2-F7" anti-CD3 antibody
DVVMTQTPVSLSVSLGSHVSISCRSSQSLVHNNGNTYLSWYLQKPGQSPQPLIYKVSNRFSGISDRFSGSGSGTDFTLEINRVEPDDLGVYYCGQGAQYPFTFGSGTKLEIK

SEQ ID NO: 107 - protein, 124 aa, Artificial Sequence
  VH of the so-called "20E5-F10" anti-CD3 antibody
EVQLVETGENLVQPGKSLRLTCATSGFSFSNAWMHWIRQSPEKQLEWVAQIKDKSNNYATYYAESVNGRFTISRDDSKSSIYLHMDNLKEEDSAIYYCRYVHYGVRFFYTMDVWGQGTSVTVSS

SEQ ID NO: 108 - protein, 15 aa, Artificial Sequence
  CDR3-H of the so-called "20E5-F10" anti-CD3 antibody
RYVHYGVRFFYTMDV

SEQ ID NO: 109 - protein, 112 aa, Artificial Sequence
  VL of the so-called "20E5-F10" anti-CD3 antibody
DVVMTQTPVSLSVSLGDQVSISCRPSQSLVHNNGNTYLSWYLQKPGQSPHPLIYKVSNRFSGISDRFSGSGSGTDFTLKISRVEPDDLGVYYCGQGTQYPFTFGSGTKLEIK

SEQ ID NO: 110 - protein, 121 aa, Artificial Sequence
  VH of the so-called "20B5-F10" anti-CD3 antibody
EVQLVETGGSLVQPGKSLKLTCATSGFTFSNAWMHWVRQSPEKQLEWVAQIKAKSNNYATYYAESVKGRFTISRDDSISSVYLQMNNLKEEDTAIYYCRGVYYGFLGMDAWGQGTSVTVSS

SEQ ID NO: 111 - protein, 12 aa, Artificial Sequence
  CDR3-H of the so-called "20B5-F10" anti-CD3 antibody
RGVYYGFLGMDA

SEQ ID NO: 112 - protein, 112 aa, Artificial Sequence
  VL of the so-called "20B5-F10" anti-CD3 antibody
DVVMTQTPVSLSVSLGGQVSISCRSSQRLVHNNGNTYLSWYLQKPGQSPQLLVYKVSNRFSGISDRFSGSGSGTDFTLKISRVEPDDLGVYYCGQGTEYPFTFGSGTKLEIK

SEQ ID NO: 113 - protein, 11 aa, Artificial Sequence
  CDR1-L of the so-called "20B5-F10" anti-CD3 antibody
QRLVHNNGNTY

SEQ ID NO: 114 - protein, 9 aa, Artificial Sequence
  CDR3-L of the so-called "20B5-F10" anti-CD3 antibody
GQGTEYPFT

SEQ ID NO: 115 - protein, 119 aa, Artificial Sequence
  VH of the so-called "6C9-C9" anti-CD3 antibody
AVQLVESGGGLVRPKESLKISCAASGFTFRNAAMYWVRQAPGKGLEWVARIRTQPNNYAKYYADSVKDRFTISRDDSKSMVYLQMDNLKTEDTAMYYCTGLVVTAMDAWGQGTSVTVSS

SEQ ID NO: 116 - protein, 8 aa, Artificial Sequence
  CDR1-H of the so-called "6C9-C9" anti-CD3 antibody
GFTFRNAA

SEQ ID NO: 117 - protein, 10 aa, Artificial Sequence
  CDR2-H of the so-called "6C9-C9" anti-CD3 antibody
IRTQPNNYAK

SEQ ID NO: 118 - protein, 10 aa, Artificial Sequence
  CDR3-H of the so-called "6C9-C9" anti-CD3 antibody
TGLVVTAMDA

SEQ ID NO: 119 - protein, 106 aa, Artificial Sequence
  VL of the so-called "6C9-C9" anti-CD3 antibody
DIQMTQSPSFLSASVGDRVTINCKASQNINKYLNWYQQKLGEAPKLLIYVTNNLQTGIPSRFSGSGSGTDYTLTISSLQPEDVATYFCLQHRSMYTFGTGTKLELK

SEQ ID NO: 120 - protein, 8 aa, Artificial Sequence
  CDR3-L of the so-called "6C9-C9" anti-CD3 antibody
LQHRSMYT

SEQ ID NO: 121 - protein, 118 aa, Artificial Sequence
  VH the so-called "3E8-G1" anti-CD3 antibody
EVQVVESGGGLVQPGRSLKLSCAASGFTFSNYYMDWVRQAPKKGLEWVATITASGSRIYYPDSVKGRFTISRDNAKSSLYLLMNSLKSEDTATYYCARERTDAYFDYWGQGVMVTVSS

SEQ ID NO: 122 - protein, 8 aa, Artificial Sequence
  CDR1-H of the so-called "3E8-G1" anti-CD3 antibody
GFTFSNYY

SEQ ID NO: 123 - protein, 8 aa, Artificial Sequence
  CDR2-H of the so-called "3E8-G1" anti-CD3 antibody
ITASGSRI

SEQ ID NO: 124 - protein, 11 aa, Artificial Sequence
  CDR3-H of the so-called "3E8-G1" anti-CD3 antibody
ARERTDAYFDY

SEQ ID NO: 125 - protein, 111 aa, Artificial Sequence
  VL of the so-called "3E8-G1" anti-CD3 antibody
QFILTQPNSVSTILGSTVKLSCKRSTGNIGTNYVSWYQHHEGRSPTTMIYRDDKRPDGVPDRFSGSIDRSSNSALLTINNVQTEDEADYFCQSYISGLNPVFGGGSKLTVL

SEQ ID NO: 126 - protein, 8 aa, Artificial Sequence
  CDR1-L of the so-called "3E8-G1" anti-CD3 antibody
TGNIGTNY

SEQ ID NO: 127 - protein, 10 aa, Artificial Sequence
  CDR3-L of the so-called "3E8-G1" anti-CD3 antibody
QSYISGLNPV

SEQ ID NO: 128 - protein, 124 aa, Artificial Sequence
  VH of the so-called "3H6-D2" anti-CD3 antibody.
EVQLVETGGRLVQPGKSLKLTCATSGFTFSNAWMHWVRQSPEKQLEWVAQIKDKSNNYATYYAESVKGRFTISRDDSKSIIYLQMNSLKEEDTAIYYCRALTYYGYKRDAMDGWGHGTSVTVSS

SEQ ID NO: 129 - protein, 15 aa, Artificial Sequence
  CDR3-H of the so-called "3H6-D2" anti-CD3 antibody
RALTYYGYKRDAMDG

SEQ ID NO: 130 - protein, 112 aa, Artificial Sequence
  VL of the so-called "3H6-D2" anti-CD3 antibody.
DVVMTQTPVSLSVSLGGQVSISCRSSQSLVHNNGNTYLSWYLQKPGQSPQLLIYKVSNRFSGISDRFSGSGSGTDFTLKISRVEPDDLGVYYCGQGTQYPFTFGAGTKLELK

SEQ ID NO: 131 - protein, 114 aa, Artificial Sequence
  VH of the so-called "8H2" anti-CD3 antibody
QIQLVQSGPELKKPGESVKISCKASGYTFTDFAMNWVKQAPGNGLKWMGWINTQTGKPTYADGFKQRFVFSLETSASTIYLQINNLNIEDTATYFCTRGALASVGQGVMVTVSS

SEQ ID NO: 132 - protein, 112 aa, Artificial Sequence
  VL of the so-called "8H2" anti-CD3 antibody
DVVMTQTPVSLSVAIGQPASISCKSSQSLVGTSGKTYLNWLLQRPGQSPKRLIYLVSKLDSGIPDRFSGSGSETDFTLKISRVETDDLGVYYCLQGSHFPLTFGSGTKLEIK

SEQ ID NO: 133 - protein, 11 aa, Artificial Sequence
  CDR1-L of the so-called "8H2" anti-CD3 antibody
QSLVGTSGKTY

SEQ ID NO: 134 - protein, 9 aa, Artificial Sequence
  CDR3-L of the so-called "8H2" anti-CD3 antibody
LQGSHFPLT

SEQ ID NO: 135 - protein, 121 aa, Artificial Sequence
  VH1a of humanized "20G6" anti-CD3 antibody
QVQLVESGGGVVQPGRSLRLSCAASGFTFTKAWMHWVRQAPGKGLEWVAQIKDKSNSYATYYADSVKGRFTISRDNSKNTLYLQMNSLRAEDTAVYYCRGVYYALSPFDYWGQGTLVTVSS

SEQ ID NO: 136 - protein, 121 aa, Artificial Sequence
  VH1b of humanized "20G6" anti-CD3 antibody.
QVQLVESGGGVVQPGRSLRLSCAASGFTFTKAWMHWVRQAPGKQLEWVAQIKDKSNSYATYYADSVKGRFTISRDNSKNTLYLQMNSLRAEDTAVYYCRGVYYALSPFDYWGQGTLVTVSS

SEQ ID NO: 137 - protein, 121 aa, Artificial Sequence
  VH1c of humanized "20G6" anti-CD3 antibody.
QVQLVESGGGVVQPGRSLRLSCAASGFTFTKAWMHWVRQAPGKQLEWVAQIKDKSNSYATYYAASVKGRFTISRDDSKNTLYLQMNSLRAEDTAVYYCRGVYYALSPFDYWGQGTLVTVSS

SEQ ID NO: 138 - protein, 121 aa, Artificial Sequence
  VH1d of humanized "20G6" anti-CD3 antibody
QVQLVESGGGVVQPGRSLRLSCAASGFTFTKAWMHWVRQAPGKQLEWVAQIKDKSNSYATYYADSVKGRFTISRDDSKNTLYLQMNSLRAEDTAVYYCRGVYYALSPFDYWGQGTLVTVSS

SEQ ID NO: 139 - protein, 112 aa, Artificial Sequence
  VL1a of humanized "20G6" anti-CD3 antibody
DIVMTQTPLSLSVTPGQPASISCKSSQSLVHNNGNTYLSWYLQKPGQSPQLLIYKVSNRFSGVPDRFSGSGSGTDFTLKISRVEAEDVGVYYCGQGTQYPFTFGQGTKLEIK

SEQ ID NO: 140 - protein, 112 aa, Artificial Sequence
  VL1b of humanized "20G6" anti-CD3 antibody
DIVMTQTPLSLSVTPGQPASISCKSSQSLVHNNGNTYLSWYLQKPGQSPQLLIYKVSNRFSGVPDRFSGSGSGTDFTLKISRVEAEDVGVYYCGQGTQYPFTFGGGTKVEIK

SEQ ID NO: 141 - protein, 112 aa, Artificial Sequence
  VL1c of humanized "20G6" anti-CD3 antibody.
DIVMTQTPLSLSVTPGQPASISCKSSQSLVHNNANTYLSWYLQKPGQSPQSLIYKVSNRFSGVPDRFSGSGSGTDFTLKISRVEAEDVGVYYCGQGTQYPFTFGSGTKVEIK

SEQ ID NO: 142 - protein, 11 aa, Artificial Sequence
  CDR1-L of the VL1c variant of the humanized "20G6" anti-CD3 antibody.
QSLVHNNANTY

SEQ ID NO: 143 - protein, 112 aa, Artificial Sequence
  VL1d of humanized "20G6" anti-CD3 antibody
DIVMTQTPLSLSVTPGQPASISCKSSQSLVHNNGNTYLSWYLQKPGQSPQSLIYKVSNRFSGVPDRFSGSGSGTDFTLKISRVEAEDVGVYYCGQGTQYPFTFGSGTKVEIK

SEQ ID NO: 144 - protein, 121 aa, Artificial Sequence
  VH2a of humanized "20G6" anti-CD3 antibody
EVQLVESGGGLVQPGGSLRLSCAASGFTFTKAWMNWVRQAPGKGLEWVSQIKDKSNSYATYYADSVKGRFTISRDNAKNSLYLQMNSLRDEDTAVYYCRGVYYALSPFDYWGQGTLVTVSS

SEQ ID NO: 145 - protein, 121 aa, Artificial Sequence
  VH2b of humanized "20G6" anti-CD3 antibody.
EVQLVESGGGLVQPGGSLRLSCAASGFTFTKAWMHWVRQAPGKGLEWVSQIKDKSNSYATYYADSVKGRFTISRDNAKNSLYLQMNSLRDEDTAVYYCRGVYYALSPFDYWGQGTLVTVSS

SEQ ID NO: 146 - protein, 121 aa, Artificial Sequence
  VH2c of humanized "20G6" anti-CD3 antibody
EVQLVESGGGLVQPGGSLRLSCAASGFTFTKAWMHWVRQAPGKQLEWVSQIKDKSNSYATYYAASVKGRFTISRDDAKNSLYLQMNSLRDEDTAVYYCRGVYYALSPFDYWGQGTLVTVSS

SEQ ID NO: 147 - protein, 121 aa, Artificial Sequence
  VH2d of humanized "20G6" anti-CD3 antibody
EVQLVESGGGLVQPGGSLRLSCAASGFTFTKAWMHWVRQAPGKQLEWVSQIKDKSNSYATYYADSVKGRFTISRDDAKNSLYLQMNSLRDEDTAVYYCRGVYYALSPFDYWGQGTLVTVSS

SEQ ID NO: 148 - protein, 112 aa, Artificial Sequence
  VL2a of humanized "20G6" anti-CD3 antibody
DIVMTQSPLSLPVTPGEPASISCRSSQSLVHNNGNTYLDWYLQKPGQSPQLLIYKVSNRASGVPDRFSGSGSGTDFTLKISRVEAEDVGVYYCGQGTQYPFTFGQGTKLEIK

SEQ ID NO: 149 - protein, 112 aa, Artificial Sequence
  VL2b of humanized "20G6" anti-CD3 antibody
DIVMTQSPLSLPVTPGEPASISCRSSQSLVHNNGNTYLDWYLQKPGQSPQLLIYKVSNRASGVPDRFSGSGSGTDFTLKISRVEAEDVGVYYCGQGTQYPFTFGGGTKVEIK

SEQ ID NO: 150 - protein, 112 aa, Artificial Sequence
  VL2c of humanized "20G6" anti-CD3 antibody
DIVMTQSPLSLPVTPGEPASISCRSSQSLVHNNGNTYLDWYLQKPGQSPQLLIYKVSNRFSGVPDRFSGSGSGTDFTLKISRVEAEDVGVYYCGQGTQYPFTFGSGTKVEIK

SEQ ID NO: 151 - protein, 112 aa, Artificial Sequence
  VL2d of humanized "20G6" anti-CD3 antibody
DIVMTQSPLSLPVTPGEPASISCRSSQSLVHNNGNTYLSWYLQKPGQSPQSLIYKVSNRFSGVPDRFSGSGSGTDFTLKISRVEAEDVGVYYCGQGTQYPFTFGSGTKVEIK

SEQ ID NO: 152 - protein, 121 aa, Artificial Sequence
  VH3a of humanized "20G6" anti-CD3 antibody
QVQLVQSGAEVKKPGASVKVSCKASGFTFTKAWMHWVRQAPGQGLEWMGQIKDKSNSYATYYAQKFQGRVTMTRDTSTSTVYMELSSLRSEDTAVYYCRGVYYALSPFDYWGQGTLVTVSS

SEQ ID NO: 153 - protein, 121 aa, Artificial Sequence
  VH3b of humanized "20G6" anti-CD3 antibody
QVQLVQSGAEVKKPGASVKVSCKASGFTFTKAWMHWVRQAPGKQLEWMGQIKDKSNSYATYYAQKFQGRVTMTRDTSTSTVYMELSSLRSEDTAVYYCRGVYYALSPFDYWGQGTLVTVSS

SEQ ID NO: 154 - protein, 112 aa, Artificial Sequence
  VL3a of humanized "20G6" anti-CD3 antibody
DIVMTQSPDSLAVSLGERATINCKSSQSLVHNNGNTYLAWYQQKPGQSPKLLIYKVSNRESGVPDRFSGSGSGTDFTLTISSLQAEDVAVYYCGQGTQYPFTFGGGTKVEIK

SEQ ID NO: 155 - protein, 112 aa, Artificial Sequence
  VL3b of humanized "20G6" anti-CD3 antibody
DIVMTQSPDSLAVSLGERATINCKSSQSLVHNNGNTYLAWYQQKPGQSPKLLIYKVSNRESGVPDRFSGSGSGTDFTLTISSLQAEDVAVYYCGQGTQYPFTFGQGTKLEIK

SEQ ID NO: 156 - protein, 112 aa, Artificial Sequence
  VL3c of humanized "20G6" anti-CD3 antibody
DIVMTQSPSSLAVSLGERATINCKSSQSLVHNNGNTYLAWYQQKPGQSPKLLIYKVSNRFSGVPDRFSGSGSGTDFTLTISSLQAEDVAVYYCGQGTQYPFTFGSGTKVEIK

SEQ ID NO: 157 - protein, 112 aa, Artificial Sequence
  VL3d of humanized "20G6" anti-CD3 antibody
DIVMTQSPDSLAVSLGERATINCKSSQSLVHNNGNTYLSWYQQKPGQSPKSLIYKVSNRFSGVPDRFSGSGSGTDFTLTISSLQAEDVAVYYCGQGTQYPFTFGSGTKVEIK

SEQ ID NO: 158 - protein, 112 aa, Artificial Sequence
  VL1A of humanized "4B4" anti-CD3 antibody
DVVMTQTPVSLSVSVGGRVSISCRSSQSLVHDNGNTYLSWSLQKPGKSPKVLIYKVSNRFSGVSSRFTGSGSGTDFTLKISSVQPDDLGVYYCGQGTQYPFTFGSGTKLEIK

SEQ ID NO: 159 - protein, 112 aa, Artificial Sequence
  VL1B of humanized "4B4" anti-CD3 antibody.
DVVMTQTPVSLSVSVGGRVSISCRSSQSLVHDNANTYLSWSLQKPGKSPKVLIYKVSNRFSGVSSRFTGSGSGTDFTLKISSVQPDDLGVYYCGQGTQYPFTFGSGTKLEIK

SEQ ID NO: 160 - protein, 112 aa, Artificial Sequence
  VL2A of humanized "4B4" anti-CD3 antibody
DVVMTQTPVSLSVSPGGPVSISCRSSQSLVHDNGNTYLSWSLQKPGQSPQVLIYKVSNRFSGVSDRFTGSGSGTDFTLKISRVEPDDLGVYYCGQGTQYPFTFGSGTKLEIK

SEQ ID NO: 161 - protein, 112 aa, Artificial Sequence
  VL2B of humanized "4B4" anti-CD3 antibody
DVVMTQTPVSLSVSPGGPVSISCRSSQSLVHDNANTYLSWSLQKPGQSPQVLIYKVSNRFSGVSDRFTGSGSGTDFTLKISRVEPDDLGVYYCGQGTQYPFTFGSGTKLEIK

SEQ ID NO: 162 - protein, 112 aa, Artificial Sequence
  VL1Cmodif1 of humanized "4B4" anti-CD3 antibody
DVVMTQSPLSLPVTLGQPVSISCRSSQSLVHDNGNTYLSWSLQRPGQSPRVLIYKVSNRFSGVPDRFSGSGSGTDFTLKISRVEAEDVGVYYCGQGTQYPFTFGSGTKLEIK

SEQ ID NO: 163 - protein, 112 aa, Artificial Sequence
  VL1Cmodif2 of humanized "4B4" anti-CD3 antibody
DVVMTQSPLSLSVTLGQPVSISCRSSQSLVHDNGNTYLSWSLQRPGQSPRVLIYKVSNRFSGVPDRFSGSGSGTDFTLKISRVEAEDVGVYYCGQGTQYPFTFGSGTKLEIK

SEQ ID NO: 164 - protein, 112 aa, Artificial Sequence
  VL1Cmodif3 of humanized "4B4" anti-CD3 antibody
DVVMTQSPLSLSVTLGQPVSISCRSSQSLVHDNANTYLSWSLQRPGQSPRVLIYKVSNRFSGVPDRFSGSGSGTDFTLKISRVEAEDVGVYYCGQGTQYPFTFGSGTKLEIK

SEQ ID NO: 165 - protein, 112 aa, Artificial Sequence
  VL1Amodif1of humanized "4B4" anti-CD3 antibody
DVVMTQSPLSLPVTLGQPVSISCRSSQSLVHDNGNTYLNWFLQRPGQSPRRLIYKVSNRDSGVPDRFSGSGSGTDFTLKISRVEAEDVGVYYCGQGTQYPFTFGQGTKLEIK

SEQ ID NO: 166 - protein, 112 aa, Artificial Sequence
  VL1Amodif2of humanized "4B4" anti-CD3 antibody
DVVMTQSPLSLSVTLGQPVSISCRSSQSLVHDNGNTYLNWFLQRPGQSPRRLIYKVSNRDSGVPDRFSGSGSGTDFTLKISRVEAEDVGVYYCGQGTQYPFTFGQGTKLEIK

SEQ ID NO: 167 - protein, 112 aa, Artificial Sequence
  VL1Amodif3 of humanized "4B4" anti-CD3 antibody
DVVMTQSPLSLSVTLGQPVSISCRSSQSLVHDNGNTYLNWFLQRPGQSPRRLIYKVSNRDSGVPDRFSGSGSGTDFTLKISRVEAEDVGVYYCGQGTQYPFTFGSGTKLEIK

SEQ ID NO: 168 - protein, 112 aa, Artificial Sequence
  VL2C of humanized "4B4" anti-CD3 antibody
DIVMTQTPLSLSVTPGQPASISCKSSQSLVHDNGNTYLSWSLQKPGQSPQVLIYKVSNRFSGVPDRFSGSGSGTDFTLKISRVEAEDVGVYYCGQGTQYPFTFGSGTKLEIK

SEQ ID NO: 169 - protein, 112 aa, Artificial Sequence
  VL2D of humanized "4B4" anti-CD3 antibody
DIVMTQTPLSLSVTPGQPASISCKSSQSLVHDNGNTYLSWYLQKPGQSPQSLIYKVSNRFSGVPDRFSGSGSGTDFTLKISRVEAEDVGVYYCGQGTQYPFTFGSGTKVEIK

SEQ ID NO: 170 - protein, 112 aa, Artificial Sequence
  VL2F of humanized "4B4" anti-CD3 antibody
DIVMTQTPLSLSVTPGQPASISCKSSQSLVHDNANTYLSWYLQKPGQSPQSLIYKVSNRFSGVPDRFSGSGSGTDFTLKISRVEAEDVGVYYCGQGTQYPFTFGSGTKVEIK

SEQ ID NO: 171 - protein, 121 aa, Artificial Sequence
  VH1A of humanized "4B4" anti-CD3 antibody
QVQLVETGGGLVKPGQSLKLTCATSGFTFSNAWMHWVRQSPEKGLEWVAQIKARSNNYATYYAESVKGRFTISRDDSKSTIYLQMNSLTPEDTAIYYCRGTYYASKPFDYWGQGVMVTVSS

SEQ ID NO: 172 - protein, 121 aa, Artificial Sequence
  VH1B of humanized "4B4" anti-CD3 antibody
QVQLVETGGGLVKPGQSLKLTCATSGFTFSNAWMHWVRQSPEKGLEWVAQIKARSNNYATYYAVSVKGRFTISRDDSKSTIYLQMNSLTPEDTAIYYCRGTYYASKPFDYWGQGVMVTVSS

SEQ ID NO: 173 - protein, 121 aa, Artificial Sequence
  VH2A of humanized "4B4" anti-CD3 antibody
EVQLVETGGGLVQPGGSLKLTCATSGFTFSNAWMHWVRQSPEKGLEWVAQIKARSNNYATYYAESVKGRFTISRDDSKSTIYLQMNSLRAEDTAIYYCRGTYYASKPFDYWGQGVMVTVSS

SEQ ID NO: 174 - protein, 121 aa, Artificial Sequence
  VH2B of humanized "4B4" anti-CD3 antibody
EVQLVETGGGLVQPGGSLKLTCATSGFTFSNAWMHWVRQSPEKGLEWVAQIKARSNNYATYYADSVKGRFTISRDDSKSTIYLQMNSLRAEDTAIYYCRGTYYASKPFDYWGQGVMVTVSS

SEQ ID NO: 175 - protein, 121 aa, Artificial Sequence
  VH6Bmodif1 of humanized "4B4" anti-CD3 antibody
QVQLVESGGGVVQPGRSLRLSCAASGFTFSNAWMHWVRQAPGKQLEWVAQIKARSNNYATYYAESVKGRFTISRDDSKSTIYLQMNSLRAEDTAVYYCRGTYYASKPFDYWGQGTTVTVSS

SEQ ID NO: 176 - protein, 121 aa, Artificial Sequence
  VH6Bmodif2 of humanized "4B4" anti-CD3 antibody
QVQLVESGGRVVQPGRSLRLTCAASGFTFSNAWMHWVRQAPGKQLEWVAQIKARSNNYATYYAESVKGRFTISRDDSKSTIYLQMNSLRAEDTAVYYCRGTYYASKPFDYWGQGTTVTVSS

SEQ ID NO: 177 - protein, 121 aa, Artificial Sequence
  VH6Amodif1 of humanized "4B4" anti-CD3 antibody
QVQLVESGGGVVQPGRSLRLSCAASGFTFSNAWMHWVRQAPGKGLEWVAQIKARSNNYATYYADSVKGRFTISRDDSKSTIYLQMNSLRAEDTAVYYCRGTYYASKPFDYWGQGTTVTVSS

SEQ ID NO: 178 - protein, 121 aa, Artificial Sequence
  VH6Amodif2 of humanized "4B4" anti-CD3 antibody
QVQLVESGGRVVQPGRSLRLTCAASGFTFSNAWMHWVRQAPGKGLEWVAQIKARSNNYATYYADSVKGRFTISRDDSKSTIYLQMNSLRAEDTAVYYCRGTYYASKPFDYWGQGTTVTVSS

SEQ ID NO: 179 - protein, 121 aa, Artificial Sequence
  VH6Amodif3 of humanized "4B4" anti-CD3 antibody
QVQLVESGGRVVQPGRSLRLTCAASGFTFSNAWMHWVRQAPGKQLEWVAQIKARSNNYATYYADSVKGRFTISRDDSKSTIYLQMNSLRAEDTAVYYCRGTYYASKPFDYWGQGTTVTVSS

SEQ ID NO: 180 - protein, 121 aa, Artificial Sequence
  VH6C of humanized "4B4" anti-CD3 antibody
QVQLVESGGGVVQPGRSLRLSCAASGFTFSNAWMHWVRQAPGKQLEWVAQIKARSNNYATYYADSVKGRFTISRDDSKSTLYLQMNSLRAEDTAVYYCRGTYYASKPFDYWGQGTLVTVSS

SEQ ID NO: 181 - protein, 121 aa, Artificial Sequence
  VH6D of humanized "4B4" anti-CD3 antibody
QVQLVESGGGVVQPGRSLRLSCATSGFTFSNAWMHWVRQAPGKQLEWVAQIKARSNNYATYYADSVKGRFTISRDDSKSTIYLQMNSLRAEDTAVYYCRGTYYASKPFDYWGQGTLVTVSS

SEQ ID NO: 182 - protein, 112 aa, Artificial Sequence
  VL "D7-VK3mut" of humanized "4B4" anti-CD3 antibody
DVVMTQSPLSLPVTLGQPASISCRSSQSLVHDNGNTYLSWSQQRPGQSPRVLIYKVSNRFSGVPDRFSGSGSGTDFTLKISRVEAEDVGVYYCGQGTQYPFTFGQGTKVEIK

SEQ ID NO: 183 - protein, 121 aa, Artificial Sequence
  D7-VH1mut of humanized "4B4" anti-CD3 antibody
EVQLVESGGGLVKPGGSLRLSCATSGFTFSNAWMHWVRQAPGKGLEWVGQIKARSNNYATYYAESVKGRFTISRDDSKNTLYLQMNSLKTEDTAVYYCRGTYYASKPFDYWGQGTLVTVSS

SEQ ID NO: 184 - protein, 11 aa, Artificial Sequence
  CDR1-L of the VL1B, VL2B, VL1Cmofif3 and VL2F variants of the humanized "4B4" anti-CD3 antibody
QSLVHDNANTY

SEQ ID NO: 185 - protein, 182 aa, Homo sapiens
MEQGKGLAVLILAIILLQGTLAQSIKGNHLVKVYDYQEDGSVLLTCDAEAKNITWFKDGKMIGFLTEDKKKWNLGSNAKDPRGMYQCKGSQNKSKPLQVYYRMCQNCIELNAATISGFLFAEIVSIFVLAVGVYFIAGQDGVRQSRASDKQTLLPNDQLYQPLKDREDDQYSHLQGNQLRRN

SEQ ID NO: 186 - protein, 249 aa, Artificial Sequence
  heavy chain sequence of "20G6-F3" Fab
EVQLVETGGSLVQPGKSLKLTCATSGFTFTKAWMHWVRQSPEKQLEWVAQIKDKSNSYATYYAESVKGRFTISRDDSKSTIYLQMNSLKEEDTAIYYCRGVYYALSPFDYWGQGVMVTVSSASTKGPSVFPLAPSSKSTSGGTAALGCLVKDYFPEPVTVSWNSGALTSGVHTFPAVLQSSGLYSLSSVVTVPSSSLGTQTYICNVNHKPSNTKVDKKVEPKSCDKTHTEQKLISEEDLNGAAHHHHHH

SEQ ID NO: 187 - protein, 219 aa, Artificial Sequence
  light chain sequence of "20G6-F3" Fab
DVVMTQTPVSLSVSLGGQVSISCRSSQSLVHNNGNTYLSWYLQKPGQSPQSLIYKVSNRFSGFSDRFSGSGSGTDFTLKISRVDPDDLGVYYCGQGTQYPFTFGSGTKLEIKRTVAAPSVFIFPPSDEQLKSGTASVVCLLNNFYPREAKVQWKVDNALQSGNSQESVTEQDSKDSTYSLSSTLTLSKADYEKHKVYACEVTHQGLSSPVTKSFNRGEC

SEQ ID NO: 188 - protein, 250 aa, Artificial Sequence
  heavy chain sequence of "4E7-C9" Fab
EVQVVETGGSLVQPGKSLKLTCATSGFTFSNAWMHWVRQSPEKQLEWVAQIKDKSNNYATYYAESLKGRFTISRDDPKRSIYLQMNSLREEDTAIYYCRYVHYGIGYAMDAWGQGTSVTVSSASTKGPSVFPLAPSSKSTSGGTAALGCLVKDYFPEPVTVSWNSGALTSGVHTFPAVLQSSGLYSLSSVVTVPSSSLGTQTYICNVNHKPSNTKVDKKVEPKSCDKTHTEQKLISEEDLNGAAHHHHHH

SEQ ID NO: 189 - protein, 219 aa, Artificial Sequence
  light chain sequence of "4E7-C9" Fab
DVVMTQTPVSLSVSLGGQVSISCRSSQSLEHNNGNTYLSWYLQKPGQSPQPLIYKVSNRFSGISDRFSGSGSGTDFTLKISRVEPDDLGVYYCGQGTQYPFTFGPGTKLELKRTVAAPSVFIFPPSDEQLKSGTASVVCLLNNFYPREAKVQWKVDNALQSGNSQESVTEQDSKDSTYSLSSTLTLSKADYEKHKVYACEVTHQGLSSPVTKSFNRGEC

SEQ ID NO: 190 - protein, 249 aa, Artificial Sequence
  heavy chain sequence of "4B4-D7" Fab
EVQLVETGGRLVQPGRSLKLTCATSGFTFSNAWMHWVRQSPEKQLEWVAQIKARSNNYATYYAESVKGRFTISRDDSKSTIYLQMNSLKEEDTAIYYCRGTYYASKPFDYWGQGVMVTVSSASTKGPSVFPLAPSSKSTSGGTAALGCLVKDYFPEPVTVSWNSGALTSGVHTFPAVLQSSGLYSLSSVVTVPSSSLGTQTYICNVNHKPSNTKVDKKVEPKSCDKTHTEQKLISEEDLNGAAHHHHHH

SEQ ID NO: 191 - protein, 218 aa, Artificial Sequence
  light chain sequence of "4B4-D7 "  Fab
DVVMTQTPVSLSVSLGGQVSISCRSSQSLVHDNGNTYLSWSLQRPGQSPQVLIYKVSNRFSGTSDRFTGSGSGTDFTLKISRVEPDDLGVYYCGQGTQYPFTFGSGTKLEIKRTVAAPSVFIFPPSDEQLKSGTASVVCLLNNFYPREAKVQWKVDNALQSGNSQESVTEQDSKDSTYSLSSTLTLSKADYEKHKVYACEVTHQGLSSPVTKSFNRGE

SEQ ID NO: 192 - protein, 250 aa, Artificial Sequence
  heavy chain sequence of "18F5-H10" Fab
EVQVVETGGSLVQPGKSLKLTCATSGFTFTNAWMHWVRRSPEKQLEWVAQIKDKSNNYATYYAESVKGRFTISRDDSKSSIYLQMNSLKEEDTAIYYCRYVHYRFAYALDAWGRGTSVSVSSASTKGPSVFPLAPSSKSTSGGTAALGCLVKDYFPEPVTVSWNSGALTSGVHTFPAVLQSSGLYSLSSVVTVPSSSLGTQTYICNVNHKPSNTKVDKKVEPKSCDKTHTEQKLISEEDLNGAAHHHHHH

SEQ ID NO: 193 - protein, 219 aa, Artificial Sequence
  light chain sequence of "18F5-H10"  Fab
DVLMTQTPVSLSVSLGGQVSISCRSSQSLVHTNGNTYLSWYLQKPGQSPQLLIYKVSNRLSGISDRFSGSGSGTDFTLKISRVEPDDLGVYYCGQGTHYPFTFGAGTKLELKRTVAAPSVFIFPPSDEQLKSGTASVVCLLNNFYPREAKVQWKVDNALQSGNSQESVTEQDSKDSTYSLSSTLTLSKADYEKHKVYACEVTHQGLSSPVTKSFNRGEC

SEQ ID NO: 194 - protein, 378 aa, Homo sapiens
MVLLWLTLLLIALPCLLQTKEDPNPPITNLRMKAKAQQLTWDLNRNVTDIECVKDADYSMPAVNNSYCQFGAISLCEVTNYTVRVANPPFSTWILFPENSGKPWAGAENLTCWIHDVDFLSCSWAVGPGAPADVQYDLYLNVANRRQQYECLHYKTDAQGTRIGCRFDDISRLSSGSQSSHILVRGRSAAFGIPCTDKFVVFSQIEILTPPNMTAKCNKTHSFMHWKMRSHFNRKFRYELQIQKRMQPVITEQVRDRTSFQLLNPGTYTVQIRARERVYEFLSAWSTPQRFECDQEEGANTRAWRTSLLIALGTLLALVCVFVICRRYLVMQRLFPRIPHMKDPIGDSFQNDKLVVWEAGKAGLEECLVTEVQVVQKT

SEQ ID NO: 195 - protein, 378 aa, Macaca fascicularis
MTLLWLTLLLVATPCLLRTKEDPNAPIRNLRMKEKAQQLMWDLNRNVTDVECIKGTDYSMPAMNNSYCQFGAISLCEVTNYTVRVASPPFSTWILFPENSGTPRAGAENLTCWVHDVDFLSCSWVVGPAAPADVQYDLYLNNPNSHEQYRCLHYKTDARGTQIGCRFDDIAPLSRGSQSSHILVRGRSAAVSIPCTDKFVFFSQIERLTPPNMTGECNETHSFMHWKMKSHFNRKFRYELRIQKRMQPVRTEQVRDTTSFQLPNPGTYTVQIRARETVYEFLSAWSTPQRFECDQEEGASSRAWRTSLLIALGTLLALLCVFLICRRYLVMQRLFPRIPHMKDPIGDTFQQDKLVVWEAGKAGLEECLVSEVQVVEKT

SEQ ID NO: 196 - protein, 523 aa, Homo sapiens
  DOMAIN (1)..(284): extracellular domain of human CD123
  MISC_FEATURE (285)..(519): Strep-II tagged Fc-Fusion
TKEDPNPPITNLRMKAKAQQLTWDLNRNVTDIECVKDADYSMPAVNNSYCQFGAISLCEVTNYTVRVANPPFSTWILFPENSGKPWAGAENLTCWIHDVDFLSCSWAVGPGAPADVQYDLYLNVANRRQQYECLHYKTDAQGTRIGCRFDDISRLSSGSQSSHILVRGRSAAFGIPCTDKFVVFSQIEILTPPNMTAKCNKTHSFMHWKMRSHFNRKFRYELQIQKRMQPVITEQVRDRTSFQLLNPGTYTVQIRARERVYEFLSAWSTPQRFECDQEEGANTRAWRDKTHTCPPCPAPELLGGPSVFLFPPKPKDTLMISRTPEVTCVVVDVSHEDPEVKFNWYVDGVEVHNAKTKPREEQYNSTYRVVSVLTVLHQDWLNGKEYKCKVSNKALPAPIEKTISKAKGQPREPQVYTLPPSRDELTKNQVSLTCLVKGFYPSDIAVEWESNGQPENNYKTTPPVLDSDGSFFLYSKLTVDKSRWQQGNVFSCSVMHEALHNHYTQKSLSLSPGSAWSHPQFEK

SEQ ID NO: 197 - protein, 519 aa, Macaca fascicularis
  DOMAIN (1)..(284): extracellular domain of Macaca fascicularis CD123
  MISC_FEATURE (285)..(516): Strep-II tagged Fc-fusion
TKEDPNAPIRNLRMKEKAQQLMWDLNRNVTDVECIKGTDYSMPAMNNSYCQFGAISLCEVTNYTVRVASPPFSTWILFPENTGTPRAGAENLTCWVHDVDFLSCSWVVGPAAPADVQYDLYLNNPNSHEQYRCLHYKTDARGTQIGCRFDDIARLSRGSQSSHILVRGRSAAVSIPCTDKFVFFSQIERLTPPNMTGECNETHSFMHWKMKSHFNRKFRYELRIQKRMQPVRTEQVRDTTSFQLPNPGTYTVQIRARETVYEFLSAWSTPQRFECDQEEGASSRAWRGSGGSGDKTHTCPPCPAPELLGGPSVFLFPPKPKDTLMISRTPEVTCVVVDVSHEDPEVKFNWYVDGVEVHNAKTKPREEQYNSTYRVVSVLTVLHQDWLNGKEYKCKVSNKALPAPIEKTISKAKGQPREPQVYTLPPSRDELTKNQVSLTCLVKGFYPSDIAVEWESNGQPENNYKTTPPVLDSDGSFFLYSKLTVDKSRWQQGNVFSCSVMHEALHNHYTQKSLSLSPG

SEQ ID NO: 198 - protein, 119 aa, Artificial Sequence
  VH of the so-called "1E1-G5" anti-CD123 antibody
QVQLQESGPTLVKPGDSVKMSCKAFGYTFTDHIIHWVKQSHGKSLEWIGYINPYSGGTNYNEKFKSKATLTVDKSSSTAYMEFSRLTSEDSAICYCALNYGSYYAMDAWGQGTSVTVSS

SEQ ID NO: 199 - protein, 8 aa, Artificial Sequence
  CDR1-H of the so-called "1E1-G5" and "8B11-B7" anti-CD123 antibodies
GYTFTDHI

SEQ ID NO: 200 - protein, 8 aa, Artificial Sequence
  CDR2-H of the so-called "1E1-G5" and "6D6-B8" anti-CD123 antibodies
INPYSGGT

SEQ ID NO: 201 - protein, 12 aa, Artificial Sequence
  CDR3-H of the so-called "1E1-G5", "6D6-B8", "8B11-B7" and "9F6-G3" anti-CD123 antibodies
ALNYGSYYAMDA

SEQ ID NO: 202 - protein, 107 aa, Artificial Sequence
  VL of the so-called "1E1-G5" anti-CD123 antibody
DIQMTQSPASLSASLGQTVTIECRPSEDIYSNLAWFQQKPGSSPQLLIYDANNLADGVPSRFSGSGSGTQYSLKINSLQSEDVASYFCQQYNKYPYTFGTGTKLELK

SEQ ID NO: 203 - protein, 6 aa, Artificial Sequence
  CDR1-L of the so-called "1E1-G5" anti-CD123 antibody
EDIYSN

SEQ ID NO: 204 - protein, 9 aa, Artificial Sequence
  CDR1-L of the so-called "1E1-G5" anti-CD123 antibody
QQYNKYPYT

SEQ ID NO: 205 - protein, 119 aa, Artificial Sequence
  VH of the so-called "2B8-F3" anti-CD123 antibody
EVQLVESGGGLVQPGRSLKLSCAASGFTFSDYNMAWVRQAPKKGLEWVATILYDGGRTYYRGSVKGRFTISRDNAKSTLYLRMDSLRSEDTATYYCATHSRGTDYFDYWGQGVMVTVSS

SEQ ID NO: 206 - protein, 8 aa, Artificial Sequence
  CDR1-H of the so-called "2B8-F3" anti-CD123 antibody
GFTFSDYN

SEQ ID NO: 207 - protein, 8 aa, Artificial Sequence
  CDR2-H of the so-called "2B8-F3" anti-CD123 antibody
ILYDGGRT

SEQ ID NO: 208 - protein, 12 aa, Artificial Sequence
  CDR3-H of the so-called "2B8-F3" anti-CD123 antibody
ATHSRGTDYFDY

SEQ ID NO: 209 - protein, 106 aa, Artificial Sequence
  VL of the so-called "2B8-F3" anti-CD123 antibody
EIVLTQSPTSMTASPGEQVTITCRASSSINYMHWYQQKPGASPRPWIYETSKLASGVPDRFSGSASGTSYSLTINNMEAEDAATYYCQQWNYPSWTFGGGTKLELK

SEQ ID NO: 210 - protein, 5 aa, Artificial Sequence
  CDR1-L of the so-called "2B8-F3" anti-CD123 antibody
SSINY

SEQ ID NO: 211 - protein, 9 aa, Artificial Sequence
  CDR3-L of the so-called "2B8-F3" anti-CD123 antibody
QQWNYPSWT

SEQ ID NO: 212 - protein, 123 aa, Artificial Sequence
  VH of the so-called "2F8-D6" anti-CD123 antibody
QVQLKESGPGLVQPSQTLSLTCTVSGFSLTSYGVSWVRQPPGKGLEWIATISSAGSTYYDLVLKSRLSITRDTSKSQVFLKVHSLQTEDTAIYLCARDAPVFNYGSYNAMDSWGQGTSVTVSS

SEQ ID NO: 213 - protein, 8 aa, Artificial Sequence
  CDR1-H of the so-called "2F8-D6" anti-CD123 antibody
GFSLTSYG

SEQ ID NO: 214 - protein, 7 aa, Artificial Sequence
  CDR2-H of the so-called "2F8-D6" anti-CD123 antibody
ISSAGST

SEQ ID NO: 215 - protein, 17 aa, Artificial Sequence
  CDR3-H of the so-called "2F8-D6" anti-CD123 antibody
ARDAPVFNYGSYNAMDS

SEQ ID NO: 216 - protein, 106 aa, Artificial Sequence
  VL of the so-called "2F8-D6" anti-CD123 antibody
DIQMTQSPSFLSATVGDRVTINCKASQNINKYLNWYQQKLGEAPKRLIYNTNSLQTGIPSRFSGSGSGTDYTLTISSLQPEDVATYFCLQHKSGLTFGSGTKLEIK

SEQ ID NO: 217 - protein, 6 aa, Artificial Sequence
  CDR1-L of the so-called "2F8-D6" anti-CD123 antibody
QNINKY

SEQ ID NO: 218 - protein, 8 aa, Artificial Sequence
  CDR3-L of the so-called "2F8-D6" anti-CD123 antibody
LQHKSGLT

SEQ ID NO: 219 - protein, 125 aa, Artificial Sequence
  VH of the so-called "3B10-E6" anti-CD123 antibody
QVQLQQSGPELRRPGSSVRLSCKASGYRIKDFLIHWIKNRPEHGLEWIGWIDPEDGETKYAQKFQTKATLTADTSSNTAYMQLSSLTSEDTATYFCARWGDVYYGLMRGHVMDAWGQGTSVTVSS

SEQ ID NO: 220 - protein, 8 aa, Artificial Sequence
  CDR1-H of the so-called "3B10-E6" anti-CD123 antibody
GYRIKDFL

SEQ ID NO: 221 - protein, 8 aa, Artificial Sequence
  CDR2-H of the so-called "3B10-E6" anti-CD123 antibody
IDPEDGET

SEQ ID NO: 222 - protein, 18 aa, Artificial Sequence
  CDR3-H of the so-called "3B10-E6" anti-CD123 antibody
ARWGDVYYGLMRGHVMDA

SEQ ID NO: 223 - protein, 113 aa, Artificial Sequence
  VL of the so-called "3B10-E6" anti-CD123 antibody
DVLMTQTPVSLPVSLGGQVSISCRSSQSLVHSDGDTYLHWYLQKPGQSPQLLIYRVSNRFSGVPDRFSGSGSGTDFTLKISRVEPEDLGLYYCLQTTHFPPWTFGGGTKLEMK

SEQ ID NO: 224 - protein, 11 aa, Artificial Sequence
  CDR1-L of the so-called "3B10-E6" anti-CD123 antibody
QSLVHSDGDTY

SEQ ID NO: 225 - protein, 10 aa, Artificial Sequence
  CDR3-L of the so-called "3B10-E6" anti-CD123 antibody
LQTTHFPPWT

SEQ ID NO: 226 - protein, 118 aa, Artificial Sequence
  VH of the so-called "3E3-D3" anti-CD123 antibody
QVQLQESGPGLVQPSQTLSLTCTVSGFSLTTYDVHWVRQPPGKGLEWMGRIQNGGITDYNSALKSRLIISRDTSKSQVFLKMNSVQTEDTAMYFCAKTGSYFYAFDHWGQGTLVTVSS

SEQ ID NO: 227 - protein, 8 aa, Artificial Sequence
  CDR1-H of the so-called "3E3-D3" anti-CD123 antibody
GFSLTTYD

SEQ ID NO: 228 - protein, 7 aa, Artificial Sequence
  CDR2-H of the so-called "3E3-D3" anti-CD123 antibody
IQNGGIT

SEQ ID NO: 229 - protein, 12 aa, Artificial Sequence
  CDR3-H of the so-called "3E3-D3" anti-CD123 antibody
AKTGSYFYAFDH

SEQ ID NO: 230 - protein, 111 aa, Artificial Sequence
  VL of the so-called "3E3-D3" anti-CD123 antibody
QFVLTQPNSVSTNLGSTVKLSCKRNTGNIGSNYVNWYQQHEGRSPTTMIYRDDKRPDGVPDRFSGSIDRSSNSALLTINNVQTEDEADYFCQSYSSGINIIFGGGTKLTVL

SEQ ID NO: 231 - protein, 8 aa, Artificial Sequence
  CDR1-L of the so-called "3E3-D3" anti-CD123 antibody
TGNIGSNY

SEQ ID NO: 232 - protein, 10 aa, Artificial Sequence
  CDR3-L of the so-called "3E3-D3" anti-CD123 antibody
QSYSSGINII

SEQ ID NO: 233 - protein, 120 aa, Artificial Sequence
  VH of the so-called "5A5-B4" anti-CD123 antibody
QIQIVQSGSDVTSTCNGCGTCYFSGFSLSTTGICVSWIRQPSGKGQEWLADFCWDDGKGYNPSLKNRLSISKDTSNNQVFLKITSVDTADTATYYCARRRVYYGIYFDYWGQGVMVTVSS

SEQ ID NO: 234 - protein, 10 aa, Artificial Sequence
  CDR1-H of the so-called "5A5-B4" anti-CD123 antibody
GFSLSTTGIC

SEQ ID NO: 235 - protein, 7 aa, Artificial Sequence
  CDR2-H of the so-called "5A5-B4" anti-CD123 antibody
FCWDDGK

SEQ ID NO: 236 - protein, 13 aa, Artificial Sequence
  CDR3-H of the so-called "5A5-B4" anti-CD123 antibody
ARRRVYYGIYFDY

SEQ ID NO: 237 - protein, 106 aa, Artificial Sequence
  VL of the so-called "5A5-B4" anti-CD123 antibody
DIVMTQSPALAVSPGERVSISCRASNSVSTRMHWYQQKPGQQPKLLIYGASNLESGVPARFSGSGSGTDFTLTIDPVEADDIATYFCQQSWNDPLTFGSGTKLEIK

SEQ ID NO: 238 - protein, 6 aa, Artificial Sequence
  CDR1-L of the so-called "5A5-B4" anti-CD123 antibody
NSVSTR

SEQ ID NO: 239 - protein, 9 aa, Artificial Sequence
  CDR3-L of the so-called "5A5-B4" anti-CD123 antibody
QQSWNDPLT

SEQ ID NO: 240 - protein, 117 aa, Artificial Sequence
  VH of the so-called "6B10-E4" anti-CD123 antibody
EVQLVESGGGLVQPGRSLKLSCAASGFTFSHYNMAWVRQAPKKGLEWVATITYDDHSTYYRDSVKGRFTISRDTAKSTLYLQMDSLRSEDTATYYCARLVNYAFAYWGQGTLVTVSS

SEQ ID NO: 241 - protein, 8 aa, Artificial Sequence
  CDR1-H of the so-called "6B10-E4" anti-CD123 antibody
GFTFSHYN

SEQ ID NO: 242 - protein, 8 aa, Artificial Sequence
  CDR2-H of the so-called "6B10-E4" anti-CD123 antibody
ITYDDHST

SEQ ID NO: 243 - protein, 10 aa, Artificial Sequence
  CDR3-H of the so-called "6B10-E4" anti-CD123 antibody
ARLVNYAFAY

SEQ ID NO: 244 - protein, 106 aa, Artificial Sequence
  VL of the so-called "6B10-E4" anti-CD123 antibody
NIVMTQSPKSMSISVGDRVTMNCKASQTVGNNIAWYQQKPGLSPQLLIDYASNRYTGVPNRFTGGGYGTDFILTINSVQAEDAAFYYCQRMYNSPTFGGGTKLELK

SEQ ID NO: 245 - protein, 6 aa, Artificial Sequence
  CDR1-L of the so-called "6B10-E4" anti-CD123 antibody
QTVGNN

SEQ ID NO: 246 - protein, 8 aa, Artificial Sequence
  CDR3-L of the so-called "6B10-E4" anti-CD123 antibody
QRMYNSPT

SEQ ID NO: 247 - protein, 116 aa, Artificial Sequence
  VH of the so-called "6C10-C4" anti-CD123 antibody
EVKLQESGPSLVQPSETLSLTCTVSGFSLTSYSVHWVRQHSGKSLEWMGRMWNDGDTSYNSAFTSRLSISRDTSKGQVFLKMNSLQTEDTGTYYCARGHRTPFDYWGQGVMVTVSS

SEQ ID NO: 248 - protein, 8 aa, Artificial Sequence
  CDR1-H of the so-called "6C10-C4" anti-CD123 antibody
GFSLTSYS

SEQ ID NO: 249 - protein, 7 aa, Artificial Sequence
  CDR2-H of the so-called "6C10-C4" anti-CD123 antibody
MWNDGDT

SEQ ID NO: 250 - protein, 10 aa, Artificial Sequence
  CDR3-H of the so-called "6C10-C4" anti-CD123 antibody
ARGHRTPFDY

SEQ ID NO: 251 - protein, 113 aa, Artificial Sequence
  VL of the so-called "6C10-C4" and "9B8-G6" anti-CD123 antibodies
DIVMTQSPSSLAVSAGETVTINCKSSQSFLSSGDERNYVAWYQHKPGQSPKLLIYWASTRHSGVPDRFIGSGSGTDFTLTISSVQAEDLAIYYCQQYYDTPLTFGSGTKLEIK

SEQ ID NO: 252 - protein, 12 aa, Artificial Sequence
  CDR1-L of the so-called "6C10-C4" and "9B8-G6" anti-CD123 antibodies
QSFLSSGDERNY

SEQ ID NO: 253 - protein, 9 aa, Artificial Sequence
  CDR3-L of the so-called "6C10-C4", "9B8-G6" and "9D7-G3" anti-CD123 antibodies
QQYYDTPLT

SEQ ID NO: 254 - protein, 119 aa, Artificial Sequence
  VH of the so-called "6D6-B8" anti-CD123 antibody
QVQLQESGPTLVKPGDSVKMSCKASAYTFTDNIIHWVKQSHGKSLDWIGYINPYSGGTNYNGWFRSKATLTVDKSSSTAYMEFSRLTSDDSAIYYCALNYGSYYAMDAWGQGTSVTVSS

SEQ ID NO: 255 - protein, 8 aa, Artificial Sequence
  CDR1-H of the so-called "6D6-B8" anti-CD123 antibody
AYTFTDNI

SEQ ID NO: 256 - protein, 107 aa, Artificial Sequence
  VL of the so-called "6D6-B8" anti-CD123 antibody
DIQMTQSPASLSASLGETVTIDCRPSEDIFNNLAWYQQKPGNSPQLLIYDANSLADGVPSRFSGSGSGTQYSLMIIRLQSEDVASYFCHQYNIYPYTFGAGTKLELK

SEQ ID NO: 257 - protein, 6 aa, Artificial Sequence
  CDR1-L of the so-called "6D6-B8" anti-CD123 antibody
EDIFNN

SEQ ID NO: 258 - protein, 9 aa, Artificial Sequence
  CDR3-L of the so-called "6D6-B8" anti-CD123 antibody
HQYNIYPYT

SEQ ID NO: 259 - protein, 119 aa, Artificial Sequence
  VH of the so-called "8B11-B7" anti-CD123 antibody.
QVQLQESGPTLVNPGDSVKMSCKASGYTFTDHIIHWVKQSHGKSLEWIGYINPYSGGANYNGKFKSKATLTIDKSSSTAYMEFSRLTSGDSAIYYCALNYGSYYAMDAWGQGTSVTVSS

SEQ ID NO: 260 - protein, 8 aa, Artificial Sequence
  CDR2-H of the so-called "8B11-B7" anti-CD123 antibody
INPYSGGA

SEQ ID NO: 261 - protein, 107 aa, Artificial Sequence
  VL of the so-called  "8B11-B7" anti-CD123 antibody
DIQMTQSPASLSASLGETVTIECRTSKDIYSNLAWFQQEPGNSPQLLIYDASNLADGVPSRFSGSGSGTQYSLQINNLQSEDVASYFCHQYNNYPYTFGTGTKLELK

SEQ ID NO: 262 - protein, 6 aa, Artificial Sequence
  CDR1-L of the so-called  "8B11-B7" anti-CD123 antibody
KDIYSN

SEQ ID NO: 263 - protein, 9 aa, Artificial Sequence
  CDR3-L of the so-called  "8B11-B7" anti-CD123 antibody
HQYNNYPYT

SEQ ID NO: 264 - protein, 121 aa, Artificial Sequence
  VH of the so-called "9B8-G6" anti-CD123 antibody
EVKLQESGPSLVQSSQTLSLTCTVSGFSLTSYHIHWVRQPPGKGLEWMGVMWSDGDTSYSSALKSRLSISRDTSQSQVFLKMNSLQTEDTATYYCARGDYSSYIYLWFAYWGQGTLVTVSS

SEQ ID NO: 265 - protein, 8 aa, Artificial Sequence
  CDR1-H of the so-called "9B8-G6" and "9D7-C8" anti-CD123 antibodies
GFSLTSYH

SEQ ID NO: 266 - protein, 7 aa, Artificial Sequence
  CDR2-H of the so-called "9B8-G6" and "9D7-C8" anti-CD123 antibodies
MWSDGDT

SEQ ID NO: 267 - protein, 15 aa, Artificial Sequence
  CDR3-H of the so-called "9B8-G6" anti-CD123 antibody
ARGDYSSYIYLWFAY

SEQ ID NO: 268 - protein, 121 aa, Artificial Sequence
  VH of the so-called "9D7-C8" anti-CD123 antibody
EVKLQESGPSLVQSSQTLSLTCTVSGFSLTSYHIHWVRQTPGKGLEWMGVMWSDGDTSYNSALKSRLSISRDTSQSQVFLKMNSLQTEDTATYYCARGYYSSYLYLWFAYWGQGTLVTVSS

SEQ ID NO: 269 - protein, 15 aa, Artificial Sequence
  CDR3-H of the so-called "9D7-C8" anti-CD123 antibody
ARGYYSSYLYLWFAY

SEQ ID NO: 270 - protein, 113 aa, Artificial Sequence
  VL of the so-called "9D7-C8" anti-CD123 antibody
DIVMTQSPSSLAVSEGETVTINCKSSQSFLSSGDGKNYVAWYQYKPGQSPKLLIYWASTRQSGVPDRFIGSGSGTDFTLTISTVQAEDLAIYYCQQYYDTPLTFGSGTKLEIK

SEQ ID NO: 271 - protein, 12 aa, Artificial Sequence
  CDR1-L of the so-called "9D7-C8" anti-CD123 antibody
QSFLSSGDGKNY

SEQ ID NO: 272 - protein, 119 aa, Artificial Sequence
  VH of the so-called "9F6-G3" anti-CD123 antibody
QVQLQESGPTLVKPGDSVKMSCKASGYTFTDYIIHWVKQSHGKSLEWIGYINPYSDGTNYNEKFKSKATLTVDKSTSTAYMEFSRLTSEDSAIYFCALNYGSYYAMDAWGQGTSVTVSS

SEQ ID NO: 273 - protein, 8 aa, Artificial Sequence
  CDR1-H of the so-called "9F6-G3" anti-CD123 antibody
GYTFTDYI

SEQ ID NO: 274 - protein, 8 aa, Artificial Sequence
  CDR2-H of the so-called "9F6-G3" anti-CD123 antibody
INPYSDGT

SEQ ID NO: 275 - protein, 107 aa, Artificial Sequence
  VL of the so-called "9F6-G3" anti-CD123 antibody
DIQMTQSPASLSASLGETVTIECRPSEDIHSNVAWYQQKPGNSPQLLIYDASNLADGVPSRFSGSGSGTQYSLKINSLQSEDVASYFCHQYNIYPYTFGSGTKLELK

SEQ ID NO: 276 - protein, 6 aa, Artificial Sequence
  CDR1-L of the so-called "9F6-G3" anti-CD123 antibody
EDIHSN

SEQ ID NO: 277 - protein, 118 aa, Artificial Sequence
  VH_G45A of humanized "3E3" anti-CD123 antibody
QVQLQESGPGLVQPSQTLSLTCTVSGFSLTTYDVHWVRQPPGKGLEWMGRIQNAGITDYNSALKSRLIISRDTSKSQVFLKMNSVQTEDTAMYFCAKTGSYFYAFDHWGQGTLVTVSS

SEQ ID NO: 278 - protein, 118 aa, Artificial Sequence
  VHmDG variant of "3E3" anti-CD123 antibody
QVQLQESGPGLVQPSQTLSLTCTVSGFSLTTYDVHWVRQPPGKGLEWMGRIQDGGITDYNSALKSRLIISRDTSKSQVFLKMNSVQTEDTAMYFCAKTGSYFYAFDHWGQGTLVTVSS

SEQ ID NO: 279 - protein, 6 aa, Artificial Sequence
  CDR2-H of  VHmDG variant of "3E3" and CDR2H of humanized "3E3" anti-CD123 antibody
QDGGIT

SEQ ID NO: 280 - protein, 118 aa, Artificial Sequence
  VH1A of humanized "3E3" anti-CD123 antibody
QVQLQESGPGLVKPSETLSLTCTVSGFSLTTYDVHWIRQPPGKGLEWIGRIQNAGITDYNPSLKSRVTISRDTSKNQFSLKLSSVTAADTAVYYCAKTGSYFYAFDHWGQGTLVTVSS

SEQ ID NO: 281 - protein, 118 aa, Artificial Sequence
  VH1B of humanized "3E3" anti-CD123 antibody
QVQLQESGPGLVKPSETLSLTCTVSGFSLTTYDVHWVRQPPGKGLEWIGRIQNAGITDYNPSLKSRVTISRDTSKNQFSLKLSSVTAADTAVYFCAKTGSYFYAFDHWGQGTLVTVSS

SEQ ID NO: 282 - protein, 118 aa, Artificial Sequence
  VH1C of humanized "3E3" anti-CD123 antibody
QVQLQESGPGLVKPSETLSLTCTVSGFSLTTYDVHWIRQPPGKGLEWMGRIQNAGITDYNPSLKSRLTISRDTSKNQVSLKLSSVTAADTAVYYCAKTGSYFYAFDHWGQGTLVTVSS

SEQ ID NO: 283 - protein, 118 aa, Artificial Sequence
  VH1D of humanized "3E3" anti-CD123 antibody
QVQLQESGPGLVKPSETLSLTCTVSGFSLTTYDVHWVRQPPGKGLEWMGRIQNAGITDYNPSLKSRLTISRDTSKNQVSLKLSSVTAADTAVYFCAKTGSYFYAFDHWGQGTLVTVSS

SEQ ID NO: 284 - protein, 118 aa, Artificial Sequence
  VH1E of humanized "3E3" anti-CD123 antibody
QVQLQESGPGLVKPSETLSLTCTVSGFSLTTYDVHWVRQPPGKGLEWMGRIQNAGITDYNPSLKSRLTISRDTSKSQVSLKLSSVTAADTAVYFCAKTGSYFYAFDHWGQGTLVTVSS

SEQ ID NO: 285 - protein, 118 aa, Artificial Sequence
  VH1F of humanized "3E3" anti-CD123 antibody
QVQLQESGPGLVKPSETLSLTCTVSGFSLTTYDVHWIRQPPGKGLEWMGRIQNAGITDYNPALKSRLTISRDTSKSQVFLKLSSVTAADTAVYYCAKTGSYFYAFDHWGQGTLVTVSS

SEQ ID NO: 286 - protein, 118 aa, Artificial Sequence
  VH1G of humanized "3E3" anti-CD123 antibody
QVQLQESGPGLVKPSETLSLTCTVSGFSLTTYDVHWVRQPPGKGLEWMGRIQNAGITDYNPALKSRLTISRDTSKSQVFLKLSSVQAADTAVYFCAKTGSYFYAFDHWGQGTLVTVSS

SEQ ID NO: 287 - protein, 118 aa, Artificial Sequence
  VH1Fm1 of humanized "3E3" anti-CD123 antibody
QVQLQESGPGLVKPSETLSLTCTVSGFSLTTYDVHWIRQPPGKGLEWMGRIQNAGITDYNPALKSRLTISRDTSKSQVFLKMSSVTAADTAVYYCAKTGSYFYAFDHWGQGTLVTVSS

SEQ ID NO: 288 - protein, 118 aa, Artificial Sequence
  VH1Fm2 of humanized "3E3" anti-CD123 antibody
QVQLQESGPGLVKPSETLSLTCTVSGFSLTTYDVHWIRQPPGKGLEWMGRIQNAGITDYNPSLKSRLTISRDTSKSQVSLKMSSVTAADTAVYYCAKTGSYFYAFDHWGQGTLVTVSS

SEQ ID NO: 289 - protein, 118 aa, Artificial Sequence
  VH1Fm2DG of humanized "3E3" anti-CD123 antibody
QVQLQESGPGLVKPSETLSLTCTVSGFSLTTYDVHWIRQPPGKGLEWMGRIQDGGITDYNPSLKSRLTISRDTSKSQVSLKMSSVTAADTAVYYCAKTGSYFYAFDHWGQGTLVTVSS

SEQ ID NO: 290 - protein, 118 aa, Artificial Sequence
  VH1Dm1 of humanized "3E3" anti-CD123 antibody
QVQLQESGPGLVKPSETLSLTCTVSGFSLTTYDVHWVRQPPGKGLEWMGRIQNAGITDYNPSLKSRLTISRDTSKNQVSLKMSSVTAADTAVYFCAKTGSYFYAFDHWGQGTLVTVSS

SEQ ID NO: 291 - protein, 118 aa, Artificial Sequence
  VH1Em1 of humanized "3E3" anti-CD123 antibody
QVQLQESGPGLVKPSETLSLTCTVSGFSLTTYDVHWVRQPPGKGLEWMGRIQNAGITDYNPALKSRLTISRDTSKSQVSLKMSSVTAADTAVYFCAKTGSYFYAFDHWGQGTLVTVSS

SEQ ID NO: 292 - protein, 111 aa, Artificial Sequence
  VL1A of humanized "3E3" anti-CD123 antibody
NFVLTQPHSVSESPGKTVTISCTRNTGNIGSNYVQWYQQRPGSSPTTVIYRDDKRPSGVPDRFSGSIDSSSNSASLTISGLKTEDEADYYCQSYSSGINIIFGGGTKLTVL

SEQ ID NO: 293 - protein, 111 aa, Artificial Sequence
  VL1B of humanized "3E3" anti-CD123 antibody
NFVLTQPHSVSESPGKTVTISCTRNTGNIGSNYVNWYQQRPGSSPTTVIYRDDKRPSGVPDRFSGSIDSSSNSASLTISGLKTEDEADYFCQSYSSGINIIFGGGTKLTVL

SEQ ID NO: 294 - protein, 111 aa, Artificial Sequence
  VL1C of humanized "3E3" anti-CD123 antibody
NFVLTQPHSVSESPGKTVTISCTRNTGNIGSNYVNWYQQRPGSSPTTMIYRDDKRPSGVPDRFSGSIDSSSNSASLTISGLKTEDEADYFCQSYSSGINIIFGGGTKLTVL

SEQ ID NO: 295 - protein, 111 aa, Artificial Sequence
  VL1D of humanized "3E3" anti-CD123 antibody
NFVLTQPHSVSESPGKTVTISCTRNTGNIGSNYVNWYQQHPGSSPTTMIYRDDKRPSGVPDRFSGSIDSSSNSASLTISGLKTEDEADYFCQSYSSGINIIFGGGTKLTVL

SEQ ID NO: 296 - protein, 111 aa, Artificial Sequence
  VL1E of humanized "3E3" anti-CD123 antibody
NFVLTQPHSVSTSPGSTVTISCTRNTGNIGSNYVNWYQQRPGSSPTTMIYRDDKRPSGVPDRFSGSIDSSSNSASLTISGLKTEDEADYFCQSYSSGINIIFGGGTKLTVL

SEQ ID NO: 297 - protein, 111 aa, Artificial Sequence
  VL1F of humanized "3E3" anti-CD123 antibody
NFVLTQPHSVSTSPGSTVTISCTRNTGNIGSNYVNWYQQRPGSSPTTMIYRDDKRPSGVPDRFSGSIDSSSNSASLTISGVKTEDEADYFCQSYSSGINIIFGGGTKLTVL

SEQ ID NO: 298 - protein, 111 aa, Artificial Sequence
  VL1G of humanized "3E3" anti-CD123 antibody
NFVLTQPHSVSTSPGSTVTISCTRNTGNIGSNYVNWYQQHPGSSPTTMIYRDDKRPSGVPDRFSGSIDSSSNSASLTISGVKTEDEADYFCQSYSSGINIIFGGGTKLTVL

SEQ ID NO: 299 - protein, 111 aa, Artificial Sequence
  VL1Fm1 of humanized "3E3" anti-CD123 antibody
NFVLTQPHSVSTSPGSTVTISCTRNTGNIGSNYVNWYQQRPGSSPTTMIYRDDKRPSGVPDRFSGSIDRSSNSASLTISGVKTEDEADYFCQSYSSGINIIFGGGTKLTVL

SEQ ID NO: 300 - protein, 111 aa, Artificial Sequence
  VL1Fm2 of humanized "3E3" anti-CD123 antibody
NFVLTQPHSVSTSPGSTVTLSCTRNTGNIGSNYVNWYQQRPGSSPTTMIYRDDKRPDGVPDRFSGSIDRSSNSASLTISGVKTEDEADYFCQSYSSGINIIFGGGTKLTVL

SEQ ID NO: 301 - protein, 118 aa, Artificial Sequence
  VH2A of humanized "3E3" anti-CD123 antibody
QVQLQESGPGLVKPSETLSLTCTVSGFSLTTYDVHWVRQPPGKGLEWMGRIQNAGITDYNSALKSRLIISRDTSKSQVFLKMNSVTTADTAMYFCAKTGSYFYAFDHWGQGTLVTVSS

SEQ ID NO: 302 - protein, 118 aa, Artificial Sequence
  VH3A of humanized "3E3" anti-CD123 antibody
QVTLQESGPGLVKPSQTLSLTCTVSGFSLTTYDVHWVRQPPGKGLEWMGRIQNAGITDYNSALKSRLIISRDTSKSQVFLKMNSVDTVDTAMYFCAKTGSYFYAFDHWGQGTLVTVSS

SEQ ID NO: 303 - protein, 111 aa, Artificial Sequence
  VL2A of humanized "3E3" anti-CD123 antibody.
QFVLTQPPSVSTNPGSTVKLSCKRNTGNIGSNYVNWYQQKPGQSPTTMIYRDDKRPDGVPDRFSGSIDRSSNSALLTINNVQTEDEADYFCQSYSSGINIIFGGGTKLTVL

SEQ ID NO: 304 - protein, 111 aa, Artificial Sequence
  VL2Am1 of humanized "3E3" anti-CD123 antibody
QFVLTQPHSVSTNPGSTVKLSCKRNTGNIGSNYVNWYQQKPGQSPTTMIYRDDKRPDGVPDRFSGSIDRSSNSALLTINNVQTEDEADYFCQSYSSGINIIFGGGTKLTVL

SEQ ID NO: 305 - protein, 111 aa, Artificial Sequence
  VL2Am2 of humanized "3E3" anti-CD123 antibody.
QFVLTQPHSVSTNPGSTVKLSCKRNTGNIGSNYVNWYQQRPGSSPTTMIYRDDKRPDGVPDRFSGSIDRSSNSALLTINNVQTEDEADYFCQSYSSGINIIFGGGTKLTVL

SEQ ID NO: 306 - protein, 344 aa, Artificial Sequence
  polypeptide I of the so-called CODV-Fab "7G3 x 20G6" antibody-like binding protein
DVVMTQTPVSLSVSLGGQVSISCRSSQSLVHNNGNTYLSWYLQKPGQSPQSLIYKVSNRFSGFSDRFSGSGSGTDFTLKISRVDPDDLGVYYCGQGTQYPFTFGSGTKLEIKGQPKAAPDFVMTQSPSSLTVTAGEKVTMSCKSSQSLLNSGNQKNYLTWYLQKPGQPPKLLIYWASTRESGVPDRFTGSGSGTDFTLTISSVQAEDLAVYYCQNDYSYPYTFGGGTKLEIKTKGPSRTVAAPSVFIFPPSDEQLKSGTASVVCLLNNFYPREAKVQWKVDNALQSGNSQESVTEQDSKDSTYSLSSTLTLSKADYEKHKVYACEVTHQGLSSPVTKSFNRGEC

SEQ ID NO: 307 - protein, 7 aa, Artificial Sequence
  L1 of the so-called CODV-Fab "7G3x20G6", "7G3x4E7", "7G3x4B4", "7G3x18F5", "hz20G6x7G3", "7G3xhz4B4", "hz4B4x3E3" and CODV-Fab "hz20G6x7G3-TL4" antibody-like binding proteins
GQPKAAP

SEQ ID NO: 308 - protein, 113 aa, Artificial Sequence
  VL1 or VL2 domain of the so-called CODV-Fab "7G3x20G6", "7G3x4E7", "7G3x4B4", "7G3x18F5", "hz20G6x7G3", "7G3xhz4B4" and CODV-Fab "hz20G6x7G3-TL4" antibody-like binding proteins
DFVMTQSPSSLTVTAGEKVTMSCKSSQSLLNSGNQKNYLTWYLQKPGQPPKLLIYWASTRESGVPDRFTGSGSGTDFTLTISSVQAEDLAVYYCQNDYSYPYTFGGGTKLEIK

SEQ ID NO: 309 - protein, 5 aa, Artificial Sequence
  L2 of the so-called CODV-Fab "7G3x20G6", "7G3x4E7", "7G3x4B4", "7G3x18F5", "hz20G6x7G3", "7G3xhz4B4", "hz4B4x3E3" and CODV-Fab "hz20G6x7G3-TL4" antibody-like binding proteins
TKGPS

SEQ ID NO: 310 - protein, 107 aa, Artificial Sequence [sequence omitted]

SEQ ID NO: 311 - protein, 342 aa, Artificial Sequence
  polypeptide II of the so-called CODV-Fab "7G3 x 20G6" antibody-like binding protein
EVQLQQSGPELVKPGASVKMSCKASGYTFTDYYMKWVKQSHGKSLEWIGDIIPSNGATFYNQKFKGKATLTVDRSSSTAYMHLNSLTSEDSAVYYCTRSHLLRASWFAYWGQGTLVTVSASEVQLVETGGSLVQPGKSLKLTCATSGFTFTKAWMHWVRQSPEKQLEWVAQIKDKSNSYATYYAESVKGRFTISRDDSKSTIYLQMNSLKEEDTAIYYCRGVYYALSPFDYWGQGVMVTVSSRTASTKGPSVFPLAPSSKSTSGGTAALGCLVKDYFPEPVTVSWNSGALTSGVHTFPAVLQSSGLYSLSSVVTVPSSSLGTQTYICNVNHKPSNTKVDKKV

SEQ ID NO: 312 - protein, 120 aa, Artificial Sequence
  VH1 or VH2 domain of the so-called CODV-Fab "7G3x20G6", "7G3x4E7", "7G3x4B4", "7G3x18F5", "hz20G6x7G3", "7G3xhz4B4" and CODV-Fab "hz20G6x7G3-TL4" antibody-like binding proteins
EVQLQQSGPELVKPGASVKMSCKASGYTFTDYYMKWVKQSHGKSLEWIGDIIPSNGATFYNQKFKGKATLTVDRSSSTAYMHLNSLTSEDSAVYYCTRSHLLRASWFAYWGQGTLVTVSA

SEQ ID NO: 313 - protein, 98 aa, Artificial Sequence
  CH1 of the so-called CODV-Fab "7G3x20G6", "7G3x4E7", "7G3x4B4", "7G3x18F5", "hz20G6x7G3", "7G3xhz4B4", "hz4B4x3E3" antibody-like binding proteins
ASTKGPSVFPLAPSSKSTSGGTAALGCLVKDYFPEPVTVSWNSGALTSGVHTFPAVLQSSGLYSLSSVVTVPSSSLGTQTYICNVNHKPSNTKVDKKV

SEQ ID NO: 314 - protein, 344 aa, Artificial Sequence
  polypeptide I of the so-called CODV-Fab "7G3 x 4E7" antibody-like binding protein
DVVMTQTPVSLSVSLGGQVSISCRSSQSLEHNNGNTYLSWYLQKPGQSPQPLIYKVSNRFSGISDRFSGSGSGTDFTLKISRVEPDDLGVYYCGQGTQYPFTFGPGTKLELKGQPKAAPDFVMTQSPSSLTVTAGEKVTMSCKSSQSLLNSGNQKNYLTWYLQKPGQPPKLLIYWASTRESGVPDRFTGSGSGTDFTLTISSVQAEDLAVYYCQNDYSYPYTFGGGTKLEIKTKGPSRTVAAPSVFIFPPSDEQLKSGTASVVCLLNNFYPREAKVQWKVDNALQSGNSQESVTEQDSKDSTYSLSSTLTLSKADYEKHKVYACEVTHQGLSSPVTKSFNRGEC

SEQ ID NO: 315 - protein, 343 aa, Artificial Sequence
  polypeptide II of the so-called CODV-Fab "7G3 x 4E7" antibody-like binding protein
EVQLQQSGPELVKPGASVKMSCKASGYTFTDYYMKWVKQSHGKSLEWIGDIIPSNGATFYNQKFKGKATLTVDRSSSTAYMHLNSLTSEDSAVYYCTRSHLLRASWFAYWGQGTLVTVSASEVQVVETGGSLVQPGKSLKLTCATSGFTFSNAWMHWVRQSPEKQLEWVAQIKDKSNNYATYYAESLKGRFTISRDDPKRSIYLQMNSLREEDTAIYYCRYVHYGIGYAMDAWGQGTSVTVSSRTASTKGPSVFPLAPSSKSTSGGTAALGCLVKDYFPEPVTVSWNSGALTSGVHTFPAVLQSSGLYSLSSVVTVPSSSLGTQTYICNVNHKPSNTKVDKKV

SEQ ID NO: 316 - protein, 344 aa, Artificial Sequence
  polypeptide I of the so-called CODV-Fab "7G3 x 4B4" antibody-like binding protein
DVVMTQTPVSLSVSLGGQVSISCRSSQSLVHDNGNTYLSWSLQRPGQSPQVLIYKVSNRFSGTSDRFTGSGSGTDFTLKISRVEPDDLGVYYCGQGTQYPFTFGSGTKLEIKGQPKAAPDFVMTQSPSSLTVTAGEKVTMSCKSSQSLLNSGNQKNYLTWYLQKPGQPPKLLIYWASTRESGVPDRFTGSGSGTDFTLTISSVQAEDLAVYYCQNDYSYPYTFGGGTKLEIKTKGPSRTVAAPSVFIFPPSDEQLKSGTASVVCLLNNFYPREAKVQWKVDNALQSGNSQESVTEQDSKDSTYSLSSTLTLSKADYEKHKVYACEVTHQGLSSPVTKSFNRGEC

SEQ ID NO: 317 - protein, 342 aa, Artificial Sequence
  polypeptide II of the so-called CODV-Fab "7G3 x 4B4" antibody-like binding protein
EVQLQQSGPELVKPGASVKMSCKASGYTFTDYYMKWVKQSHGKSLEWIGDIIPSNGATFYNQKFKGKATLTVDRSSSTAYMHLNSLTSEDSAVYYCTRSHLLRASWFAYWGQGTLVTVSASEVQLVETGGRLVQPGRSLKLTCATSGFTFSNAWMHWVRQSPEKQLEWVAQIKARSNNYATYYAESVKGRFTISRDDSKSTIYLQMNSLKEEDTAIYYCRGTYYASKPFDYWGQGVMVTVSSRTASTKGPSVFPLAPSSKSTSGGTAALGCLVKDYFPEPVTVSWNSGALTSGVHTFPAVLQSSGLYSLSSVVTVPSSSLGTQTYICNVNHKPSNTKVDKKV

SEQ ID NO: 318 - protein, 344 aa, Artificial Sequence
  polypeptide I of the so-called CODV-Fab "7G3x18F5" antibody-like binding protein.
DVLMTQTPVSLSVSLGGQVSISCRSSQSLVHTNGNTYLSWYLQKPGQSPQLLIYKVSNRLSGISDRFSGSGSGTDFTLKISRVEPDDLGVYYCGQGTHYPFTFGAGTKLELKGQPKAAPDFVMTQSPSSLTVTAGEKVTMSCKSSQSLLNSGNQKNYLTWYLQKPGQPPKLLIYWASTRESGVPDRFTGSGSGTDFTLTISSVQAEDLAVYYCQNDYSYPYTFGGGTKLEIKTKGPSRTVAAPSVFIFPPSDEQLKSGTASVVCLLNNFYPREAKVQWKVDNALQSGNSQESVTEQDSKDSTYSLSSTLTLSKADYEKHKVYACEVTHQGLSSPVTKSFNRGEC

SEQ ID NO: 319 - protein, 343 aa, Artificial Sequence
  polypeptide II of the so-called CODV-Fab "7G3x18F5" antibody-like binding protein.
EVQLQQSGPELVKPGASVKMSCKASGYTFTDYYMKWVKQSHGKSLEWIGDIIPSNGATFYNQKFKGKATLTVDRSSSTAYMHLNSLTSEDSAVYYCTRSHLLRASWFAYWGQGTLVTVSASEVQVVETGGSLVQPGKSLKLTCATSGFTFTNAWMHWVRRSPEKQLEWVAQIKDKSNNYATYYAESVKGRFTISRDDSKSSIYLQMNSLKEEDTAIYYCRYVHYRFAYALDAWGRGTSVSVSSRTASTKGPSVFPLAPSSKSTSGGTAALGCLVKDYFPEPVTVSWNSGALTSGVHTFPAVLQSSGLYSLSSVVTVPSSSLGTQTYICNVNHKPSNTKVDKKV

SEQ ID NO: 320 - protein, 344 aa, Artificial Sequence
  polypeptide I of the so-called CODV-Fab "hz20G6 x 7G3" antibody-like binding protein
DFVMTQSPSSLTVTAGEKVTMSCKSSQSLLNSGNQKNYLTWYLQKPGQPPKLLIYWASTRESGVPDRFTGSGSGTDFTLTISSVQAEDLAVYYCQNDYSYPYTFGGGTKLEIKGQPKAAPDIVMTQTPLSLSVTPGQPASISCKSSQSLVHNNGNTYLSWYLQKPGQSPQSLIYKVSNRFSGVPDRFSGSGSGTDFTLKISRVEAEDVGVYYCGQGTQYPFTFGSGTKVEIKTKGPSRTVAAPSVFIFPPSDEQLKSGTASVVCLLNNFYPREAKVQWKVDNALQSGNSQESVTEQDSKDSTYSLSSTLTLSKADYEKHKVYACEVTHQGLSSPVTKSFNRGEC

SEQ ID NO: 321 - protein, 342 aa, Artificial Sequence
  polypeptide II of the so-called CODV-Fab "hz20G6 x 7G3" antibody-like binding protein
QVQLVESGGGVVQPGRSLRLSCAASGFTFTKAWMHWVRQAPGKQLEWVAQIKDKSNSYATYYADSVKGRFTISRDDSKNTLYLQMNSLRAEDTAVYYCRGVYYALSPFDYWGQGTLVTVSSSEVQLQQSGPELVKPGASVKMSCKASGYTFTDYYMKWVKQSHGKSLEWIGDIIPSNGATFYNQKFKGKATLTVDRSSSTAYMHLNSLTSEDSAVYYCTRSHLLRASWFAYWGQGTLVTVSARTASTKGPSVFPLAPSSKSTSGGTAALGCLVKDYFPEPVTVSWNSGALTSGVHTFPAVLQSSGLYSLSSVVTVPSSSLGTQTYICNVNHKPSNTKVDKKV

SEQ ID NO: 322 - protein, 344 aa, Artificial Sequence
  polypeptide I of the so-called CODV-Fab 7G3 x hz4B4" antibody-like binding protein
DVVMTQTPVSLSVSVGGRVSISCRSSQSLVHDNGNTYLSWSLQKPGKSPKVLIYKVSNRFSGVSSRFTGSGSGTDFTLKISSVQPDDLGVYYCGQGTQYPFTFGSGTKLEIKGQPKAAPDFVMTQSPSSLTVTAGEKVTMSCKSSQSLLNSGNQKNYLTWYLQKPGQPPKLLIYWASTRESGVPDRFTGSGSGTDFTLTISSVQAEDLAVYYCQNDYSYPYTFGGGTKLEIKTKGPSRTVAAPSVFIFPPSDEQLKSGTASVVCLLNNFYPREAKVQWKVDNALQSGNSQESVTEQDSKDSTYSLSSTLTLSKADYEKHKVYACEVTHQGLSSPVTKSFNRGEC

SEQ ID NO: 323 - protein, 342 aa, Artificial Sequence
  polypeptide II of the so-called CODV-Fab "7G3 x hz4B4" antibody-like binding protein
EVQLQQSGPELVKPGASVKMSCKASGYTFTDYYMKWVKQSHGKSLEWIGDIIPSNGATFYNQKFKGKATLTVDRSSSTAYMHLNSLTSEDSAVYYCTRSHLLRASWFAYWGQGTLVTVSASQVQLVETGGGLVKPGQSLKLTCATSGFTFSNAWMHWVRQSPEKGLEWVAQIKARSNNYATYYAESVKGRFTISRDDSKSTIYLQMNSLTPEDTAIYYCRGTYYASKPFDYWGQGVMVTVSSRTASTKGPSVFPLAPSSKSTSGGTAALGCLVKDYFPEPVTVSWNSGALTSGVHTFPAVLQSSGLYSLSSVVTVPSSSLGTQTYICNVNHKPSNTKVDKKV

SEQ ID NO: 324 - protein, 342 aa, Artificial Sequence
  polypeptide I of the so-called CODV-Fab "hz4B4 x 3E3" antibody-like binding protein
QFVLTQPNSVSTNLGSTVKLSCKRNTGNIGSNYVNWYQQHEGRSPTTMIYRDDKRPDGVPDRFSGSIDRSSNSALLTINNVQTEDEADYFCQSYSSGINIIFGGGTKLTVLGQPKAAPDVVMTQTPVSLSVSVGGRVSISCRSSQSLVHDNGNTYLSWSLQKPGKSPKVLIYKVSNRFSGVSSRFTGSGSGTDFTLKISSVQPDDLGVYYCGQGTQYPFTFGSGTKLEIKTKGPSRTVAAPSVFIFPPSDEQLKSGTASVVCLLNNFYPREAKVQWKVDNALQSGNSQESVTEQDSKDSTYSLSSTLTLSKADYEKHKVYACEVTHQGLSSPVTKSFNRGEC

SEQ ID NO: 325 - protein, 340 aa, Artificial Sequence
  polypeptide II of the so-called CODV-Fab "hz4B4 x 3E3" antibody-like binding protein
QVQLVETGGGLVKPGQSLKLTCATSGFTFSNAWMHWVRQSPEKGLEWVAQIKARSNNYATYYAESVKGRFTISRDDSKSTIYLQMNSLTPEDTAIYYCRGTYYASKPFDYWGQGVMVTVSSSQVQLQESGPGLVQPSQTLSLTCTVSGFSLTTYDVHWVRQPPGKGLEWMGRIQNGGITDYNSALKSRLIISRDTSKSQVFLKMNSVQTEDTAMYFCAKTGSYFYAFDHWGQGTLVTVSSRTASTKGPSVFPLAPSSKSTSGGTAALGCLVKDYFPEPVTVSWNSGALTSGVHTFPAVLQSSGLYSLSSVVTVPSSSLGTQTYICNVNHKPSNTKVDKKV

SEQ ID NO: 326 - protein, 572 aa, Artificial Sequence
  polypeptide I of the so-called CODV-Fab "hz20G6 x 7G3 TL4" antibody-like binding protein
DFVMTQSPSSLTVTAGEKVTMSCKSSQSLLNSGNQKNYLTWYLQKPGQPPKLLIYWASTRESGVPDRFTGSGSGTDFTLTISSVQAEDLAVYYCQNDYSYPYTFGGGTKLEIKGQPKAAPDIVMTQTPLSLSVTPGQPASISCKSSQSLVHNNGNTYLSWYLQKPGQSPQSLIYKVSNRFSGVPDRFSGSGSGTDFTLKISRVEAEDVGVYYCGQGTQYPFTFGSGTKVEIKTKGPSRTVAAPSVFIFPPSDEQLKSGTASVVCLLNNFYPREAKVQWKVDNALQSGNSQESVTEQDSKDSTYSLSSTLTLSKADYEKHKVYACEVTHQGLSSPVTKSFNRGECESKYGPPCPPCPAPEFEGGPSVFLFPPKPKDTLMISRTPEVTCVVVDVSQEDPEVQFNWYVDGVEVHNAKTKPREEQFNSTYRVVSVLTVLHQDWLNGKEYKCKVSNKGLPSSIEKTISKAKGQPREPQVYTLPPSQEEMTKNQVSLTCLVKGFYPSDIAVEWESNGQPENNYKTTPPVLDSDGSFFLYSRLTVDKSRWQEGNVFSCSVMHEALHNRFTQKSLSLSLG

SEQ ID NO: 327 - protein, 228 aa, Artificial Sequence
  amino acid sequence Fc2 of the so-called CODV-Fab "hz20G6x7G3-TL4" antibody-like binding protein
ESKYGPPCPPCPAPEFEGGPSVFLFPPKPKDTLMISRTPEVTCVVVDVSQEDPEVQFNWYVDGVEVHNAKTKPREEQFNSTYRVVSVLTVLHQDWLNGKEYKCKVSNKGLPSSIEKTISKAKGQPREPQVYTLPPSQEEMTKNQVSLTCLVKGFYPSDIAVEWESNGQPENNYKTTPPVLDSDGSFFLYSRLTVDKSRWQEGNVFSCSVMHEALHNRFTQKSLSLSLG

SEQ ID NO: 328 - protein, 570 aa, Artificial Sequence
  polypeptide III of the so-called CODV-Fab "hz20G6 x 7G3 TL4" antibody-like binding protein
QVQLVESGGGVVQPGRSLRLSCAASGFTFTKAWMHWVRQAPGKQLEWVAQIKDKSNSYATYYADSVKGRFTISRDDSKNTLYLQMNSLRAEDTAVYYCRGVYYALSPFDYWGQGTLVTVSSSEVQLQQSGPELVKPGASVKMSCKASGYTFTDYYMKWVKQSHGKSLEWIGDIIPSNGATFYNQKFKGKATLTVDRSSSTAYMHLNSLTSEDSAVYYCTRSHLLRASWFAYWGQGTLVTVSARTASTKGPSVFPLAPCSRSTSESTAALGCLVKDYFPEPVTVSWNSGALTSGVHTFPAVLQSSGLYSLSSVVTVPSSSLGTKTYTCNVDHKPSNTKVDKRVESKYGPPCPPCPAPEFEGGPSVFLFPPKPKDTLMISRTPEVTCVVVDVSQEDPEVQFNWYVDGVEVHNAKTKPREEQFNSTYRVVSVLTVLHQDWLNGKEYKCKVSNKGLPSSIEKTISKAKGQPREPQVYTLPPSQEEMTKNQVSLTCLVKGFYPSDIAVEWESNGQPENNYKTTPPVLDSDGSFFLYSRLTVDKSRWQEGNVFSCSVMHEALHNHYTQKSLSLSLG

SEQ ID NO: 329 - protein, 97 aa, Artificial Sequence
  CH1 of the so-called CODV-Fab "hz20G6x7G3-TL4"antibody-like binding protein
ASTKGPSVFPLAPCSRSTSESTAALGCLVKDYFPEPVTVSWNSGALTSGVHTFPAVLQSSGLYSLSSVVTVPSSSLGTKTYTCNVDHKPSNTKVDKR

SEQ ID NO: 330 - protein, 229 aa, Artificial Sequence
  Fc of the so-called CODV-Fab "hz20G6x7G3-TL4"antibody-like binding protein
VESKYGPPCPPCPAPEFEGGPSVFLFPPKPKDTLMISRTPEVTCVVVDVSQEDPEVQFNWYVDGVEVHNAKTKPREEQFNSTYRVVSVLTVLHQDWLNGKEYKCKVSNKGLPSSIEKTISKAKGQPREPQVYTLPPSQEEMTKNQVSLTCLVKGFYPSDIAVEWESNGQPENNYKTTPPVLDSDGSFFLYSRLTVDKSRWQEGNVFSCSVMHEALHNHYTQKSLSLSLG

SEQ ID NO: 331 - protein, 8 aa, Artificial Sequence
  Consensus sequence  CDR1-H of anti-CD3 antibodies
  MISC_FEATURE (3)..(3): Xaa is T or S
  MISC_FEATURE (4)..(4): Xaa is F or V
  MISC_FEATURE (5)..(5): Xaa is S or T
  MISC_FEATURE (6)..(6): Xaa is N, K, L or Y
GFXXXXAW

SEQ ID NO: 332 - protein, 10 aa, Artificial Sequence
  Consensus sequence for CDR2-H of anti-CD3 antibodies
  MISC_FEATURE (3)..(3): Xaa is A or D
  MISC_FEATURE (4)..(4): Xaa is K or R
  MISC_FEATURE (5)..(5): Xaa is S or A
  MISC_FEATURE (7)..(7): Xaa is N or S
  MISC_FEATURE (9)..(9): Xaa is A or E
IKXXXNXYXT

SEQ ID NO: 333 - protein, 15 aa, Artificial Sequence
  Consensus sequence for CDRF-H of anti-CD3 antibodies
  MISC_FEATURE (2)..(2): Xaa is Y or G
  MISC_FEATURE (2)..(2): Xaa is Y, G or A
  MISC_FEATURE (3)..(3): Xaa is V, T or L
  MISC_FEATURE (4)..(4): Xaa is H, N, Y or Q
  MISC_FEATURE (6)..(6): Xaa is G, R or A
  MISC_FEATURE (7)..(7): Xaa is F or V or no amino acid
  MISC_FEATURE (8)..(8): Xaa is R or no amino acid
  MISC_FEATURE (9)..(9): Xaa is F, S or I or no amino acid
  MISC_FEATURE (10)..(10): Xaa is F, L, N, M, Y, S, A or G
  MISC_FEATURE (11)..(11): Xaa is  Y, A, K, S, N, T, F or L
  MISC_FEATURE (12)..(12): Xaa is  A, P, G or T
  MISC_FEATURE (13)..(13): Xaa is  M, L, F or S
  MISC_FEATURE (15)..(15): Xaa is A, V, Y or G
  MISC_FEATURE (15)..(15): Xaa is A, V or Y
RXXXYXXXXXXXXDX

SEQ ID NO: 334 - protein, 11 aa, Artificial Sequence
  Consensus sequence for CDR1-L of anti-CD3 antibodies
  MISC_FEATURE (2)..(2): Xaa is R or S
  MISC_FEATURE (4)..(4): Xaa is V or E
  MISC_FEATURE (6)..(6): Xaa is N, D or T
  MISC_FEATURE (9)..(9): Xaa is N or Y
QXLXHXNGXTY

SEQ ID NO: 335 - protein, 9 aa, Artificial Sequence
  consensus sequence for CDR3-L of anti-CD3 antibodies
  MISC_FEATURE (4)..(4): Xaa is T, A or S
  MISC_FEATURE (5)..(5): Xaa is H, E or Q
GQGXXYPFT

SEQ ID NO: 336 - protein, 8 aa, Artificial Sequence
  Consensus sequence for CDR1-H of the so-called "1E1-G5", "6D6-B8", "8B11-B7", "9F6-G3" anti-CD123 antibodies
  MISC_FEATURE (1)..(1): Xaa is G or A
  MISC_FEATURE (7)..(7): Xaa is H, Y or N
XYTFTDXI

SEQ ID NO: 337 - protein, 8 aa, Artificial Sequence
  consensus sequence for CDR2-H of the so-called "1E1-G5", "6D6-B8", "8B11-B7", "9F6-G3" anti-CD123 antibodies
  MISC_FEATURE (6)..(6): Xaa is G or D
  MISC_FEATURE (8)..(8): Xaa is T or A
INPYSXGX

SEQ ID NO: 338 - protein, 6 aa, Artificial Sequence
  consensus sequence for CDR1-L of the so-called "1E1-G5", "6D6-B8", "8B11-B7", "9F6-G3" anti-CD123 antibodies
  MISC_FEATURE (1)..(1): Xaa is E or K
  MISC_FEATURE (4)..(4): Xaa is F, H or Y
  MISC_FEATURE (5)..(5): Xaa is N or S
XDIXXN

SEQ ID NO: 339 - protein, 9 aa, Artificial Sequence
  consensus sequence for CDR3-L of the so-called "1E1-G5", "6D6-B8", "8B11-B7", "9F6-G3" anti-CD123 antibodies
  MISC_FEATURE (1)..(1): Xaa is H or Q
  MISC_FEATURE (5)..(5): Xaa is I, K or N
XQYNXYPYT

SEQ ID NO: 340 - protein, 8 aa, Artificial Sequence
  consensus sequence for CDR1-H of the so-called "6C10-C4", 9B8-G6", "9D7-C8" anti-CD123 antibodies
  MISC_FEATURE (8)..(8): Xaa is H or S
GFSLTSYX

SEQ ID NO: 341 - protein, 7 aa, Artificial Sequence
  Consensus sequence for CDR2-H of the so-called "1E1-G5", "6D6-B8", "8B11-B7", "9F6-G3" anti-CD123 antibodies
  misc_feature (3)..(3): Xaa can be any naturally occurring amino acid
MWXDGDT

SEQ ID NO: 342 - protein, 15 aa, Artificial Sequence
  consensus sequence for CDR3-H of the so-called "1E1-G5", "6D6-B8", "8B11-B7", "9F6-G3" anti-CD123 antibodies
  MISC_FEATURE (4)..(4): Xaa is D, Y or H
  MISC_FEATURE (5)..(5): Xaa is Y or R
  MISC_FEATURE (6)..(6): Xaa is S or T
  MISC_FEATURE (7)..(7): Xaa is S or P
  MISC_FEATURE (8)..(8): Xaa is Y or no amino acid
  MISC_FEATURE (9)..(9): Xaa is L, I or no amino acid
  MISC_FEATURE (10)..(10): Xaa is Y or no amino acid
  MISC_FEATURE (11)..(11): Xaa is L or no amino acid
  MISC_FEATURE (12)..(12): Xaa s W or no amino acid
  MISC_FEATURE (14)..(14): Xaa is A or D
ARGXXXXXXXXXFXY

SEQ ID NO: 343 - protein, 12 aa, Artificial Sequence
  Consensus sequence for CDR1-L of "1E1-G5", "6D6-B8", "8B11-B7","9F6-G3" anti-CD123 antibodies
  MISC_FEATURE (9)..(9): Xaa is E or G
  MISC_FEATURE (10)..(10): Xaa is R or K
QSFLSSGDXXNY

SEQ ID NO: 344 - protein, 5 aa, Artificial Sequence
  amino acid sequence of a linker sequence
GGGGS

SEQ ID NO: 345 - protein, 10 aa, Artificial Sequence
  amino acid sequence of a linker sequence
GGGGSGGGGS

SEQ ID NO: 346 - protein, 5 aa, Artificial Sequence
  amino acid sequence of a linker sequence
TVAAP

SEQ ID NO: 347 - protein, 5 aa, Artificial Sequence
  amino acid sequence of a linker sequence
QPKAA

SEQ ID NO: 348 - protein, 5 aa, Artificial Sequence
  amino acid sequence of a linker sequence
QRIEG

SEQ ID NO: 349 - protein, 7 aa, Artificial Sequence
  amino acid sequence of a linker sequence
ASTKGPS

SEQ ID NO: 350 - protein, 7 aa, Artificial Sequence
  amino acid sequence of a linker sequence
ASTKGPS

SEQ ID NO: 351 - protein, 7 aa, Artificial Sequence
  amino acid sequence of a linker sequence
HIDSPNK

SEQ ID NO: 352 - protein, 16 aa, Artificial Sequence
  linker and Histag sequence
EPKSCDKTHTHHHHHH

SEQ ID NO: 353 - protein, 7 aa, Artificial Sequence
  CDR2-H variant of the so-called "3E3" anti-CD123 antibody.
IQNAGIT

SEQ ID NO: 354 - protein, 4 aa, Artificial Sequence
  amino acid sequence of a linker sequence
GGGS

SEQ ID NO: 355 - protein, 5 aa, Artificial Sequence
  shows the amino acid sequence of a linker sequence
SGGGS

SEQ ID NO: 356 - protein, 7 aa, Artificial Sequence
  amino acid sequence of a linker sequence
GSGGGGS

SEQ ID NO: 357 - protein, 8 aa, Artificial Sequence
  amino acid sequence of a linker sequence
GGSGGGGS

SEQ ID NO: 358 - protein, 9 aa, Artificial Sequence
  amino acid sequence of a linker sequence
GGGSGGGGS

SEQ ID NO: 359 - protein, 4 aa, Artificial Sequence
  amino acid sequence of a linker sequence
KTHT

SEQ ID NO: 360 - protein, 5 aa, Artificial Sequence
  amino acid sequence of a linker sequence
KTHTS

SEQ ID NO: 361 - protein, 6 aa, Artificial Sequence
  amino acid sequence of a linker sequence
DKTHTS

SEQ ID NO: 362 - protein, 7 aa, Artificial Sequence
  amino acid sequence of a linker sequence
DKTHTSP

SEQ ID NO: 363 - protein, 8 aa, Artificial Sequence
  amino acid sequence of a linker sequence
SDKTHTSP

SEQ ID NO: 364 - protein, 9 aa, Artificial Sequence
  amino acid sequence of a linker sequence
SDKTHTSPP

SEQ ID NO: 365 - protein, 11 aa, Artificial Sequence
  amino acid sequence of a linker sequence
KSDKTHTSPPS

SEQ ID NO: 366 - protein, 12 aa, Artificial Sequence
  amino acid sequence of a linker sequence
PKSDKTHTSPPS

SEQ ID NO: 367 - protein, 13 aa, Artificial Sequence
  amino acid sequence of a linker sequence
PKSDKTHTSPPSP

SEQ ID NO: 368 - protein, 14 aa, Artificial Sequence
  amino acid sequence of a linker sequence
EPKSDKTHTSPPSP

SEQ ID NO: 369 - protein, 15 aa, Artificial Sequence
  the amino acid sequence of a linker sequence
EPKSDKTHTSPPSPG

SEQ ID NO: 370 - protein, 16 aa, Artificial Sequence
  amino acid sequence of a linker sequence
GEPKSDKTHTSPPSPG

SEQ ID NO: 371 - protein, 17 aa, Artificial Sequence
  amino acid sequence of a linker sequence
GEPKSDKTHTSPPSPGG

SEQ ID NO: 372 - protein, 18 aa, Artificial Sequence
  amino acid sequence of a linker sequence
GGEPKSDKTHTSPPSPGG

SEQ ID NO: 373 - protein, 19 aa, Artificial Sequence
  amino acid sequence of a linker sequence
GGEPKSDKTHTSPPSPGGG

SEQ ID NO: 374 - protein, 20 aa, Artificial Sequence
  amino acid sequence of a linker sequence
GGGEPKSDKTHTSPPSPGGG

SEQ ID NO: 375 - protein, 8 aa, Artificial Sequence
  CDR1-H of the so-called "7G3" antibody.
GYTFTDYY

SEQ ID NO: 376 - protein, 8 aa, Artificial Sequence
  CDR2-H of the so-called "7G3" antibody.
IIPSNGAT

SEQ ID NO: 377 - protein, 13 aa, Artificial Sequence
  CDR3-H of the so-called "7G3" antibody.
TRSHLLRASWFAY

SEQ ID NO: 378 - protein, 12 aa, Artificial Sequence
  CDR1-L of the so-called "7G3" antibody.
QSLLNSGNQKNY

SEQ ID NO: 379 - protein, 9 aa, Artificial Sequence
  CDR3-L of the so-called "7G3" antibody.
QNDYSYPYT

SEQ ID NO: 380 - protein, 120 aa, Artificial Sequence [sequence omitted]

SEQ ID NO: 381 - protein, 8 aa, Artificial Sequence
  CDR1-H of the so-called humanized "7G3" antibody
GYSFTDYY

SEQ ID NO: 382 - protein, 13 aa, Artificial Sequence
  CDR3-H of the so-called humanized "7G3" antibody.
ARSHLLRASWFAY

SEQ ID NO: 383 - protein, 120 aa, Artificial Sequence [sequence omitted]

SEQ ID NO: 384 - protein, 8 aa, Artificial Sequence
  CDR2-H of one of the so-called humanized "7G3" antibody.
IIPSSGAT

SEQ ID NO: 385 - protein, 113 aa, Artificial Sequence [sequence omitted]

SEQ ID NO: 386 - protein, 272 aa, Artificial Sequence
  SEQ ID NO:1 of WO2015/026892
QAVVTQEPSLTVSPGGTVTLTCRSSTGAVTTSNYANWVQQKPGQAPRGLIGGTNKRAPWTPARFSGSLLGGKAALTITGAQAEDEADYYCALWYSNLWVFGGGTKLTVLGGGGSGGGGEVQLVQSGAELKKPGASVKVSCKASGYTFTDYYMKWVRQAPGQGLEWIGDIIPSNGATFYNQKFKGRVTITVDKSTSTAYMELSSLRSEDTAVYYCARSHLLRASWFAYWGQGTLVTVSSGGCGGGEVAALEKEVAALEKEVAALEKEVAALEK

SEQ ID NO: 387 - protein, 280 aa, Artificial Sequence
  SEQ ID NO:3 of WO2015/026892
DFVMTQSPDSLAVSLGERVTMSCKSSQSLLNSGNQKNYLTWYQQKPGQPPKLLIYWASTRESGVPDRFSGSGSGTDFTLTISSLQAEDVAVYYCQNDYSYPYTFGQGTKLEIKGGGSGGGGEVQLVESGGGLVQPGGSLRLSCAASGFTFSTYAMNWVRQAPGKGLEWVGRIRSKYNNYATYYADSVKDRFTISRDDSKNSLYLQMNSLKTEDTAVYYCVRHGNFGNSYVSWFAYWGQGTLVTVSSGGCGGGKVAALKEKVAALKEKVAALKEKVAALKE

SEQ ID NO: 388 - protein, 352 aa, Artificial Sequence
  polypeptide I of the so-called CODV-Fab "hz20G6xhz7G3", CODV-Fab-OL1 "hz20G6xhz7G3" and CODV-Fab-OL1a "hz20G6xhz7G3" antibody-like binding proteins
DIVMTQSPDSLAVSLGERATINCESSQSLLNSGNQKNYLTWYQQKPGQPPKPLIYWASTRESGVPDRFSGSGSGTDFTLTISSLQAEDVAVYYCQNDYSYPYTFGQGTKLEIKGGSGSSGSGGDIVMTQTPLSLSVTPGQPASISCKSSQSLVHNNANTYLSWYLQKPGQSPQSLIYKVSNRFSGVPDRFSGSGSGTDFTLKISRVEAEDVGVYYCGQGTQYPFTFGSGTKVEIKGGSGSSGSGGRTVAAPSVFIFPPSDEQLKSGTASVVCLLNNFYPREAKVQWKVDNALQSGNSQESVTEQDSKDSTYSLSSTLTLSKADYEKHKVYACEVTHQGLSSPVTKSFNRGEC

SEQ ID NO: 389 - protein, 10 aa, Artificial Sequence
  Linker
GGSGSSGSGG

SEQ ID NO: 390 - protein, 339 aa, Artificial Sequence
  polypeptide II of the so-called CODV-Fab "hz20G6xhz7G3" antibody-like binding protein
QVQLVESGGGVVQPGRSLRLSCAASGFTFTKAWMHWVRQAPGKQLEWVAQIKDKSNSYATYYADSVKGRFTISRDDSKNTLYLQMNSLRAEDTAVYYCRGVYYALSPFDYWGQGTLVTVSSEVQLVQSGAEVKKPGESLKISCKGSGYSFTDYYMKWARQMPGKGLEWMGDIIPSSGATFYNQKFKGQVTISADKSISTTYLQWSSLKASDTAMYYCARSHLLRASWFAYWGQGTMVTVSSASTKGPSVFPLAPSSKSTSGGTAALGCLVKDYFPEPVTVSWNSGALTSGVHTFPAVLQSSGLYSLSSVVTVPSSSLGTQTYICNVNHKPSNTKVDKKV

SEQ ID NO: 391 - protein, 578 aa, Artificial Sequence
  polypeptide IV of the so-called CODV-Fab-TL1 "hz20G6xhz7G3" antibody-like binding protein
DIVMTQSPDSLAVSLGERATINCESSQSLLNSGNQKNYLTWYQQKPGQPPKPLIYWASTRESGVPDRFSGSGSGTDFTLTISSLQAEDVAVYYCQNDYSYPYTFGQGTKLEIKGGSGSSGSGGDIVMTQTPLSLSVTPGQPASISCKSSQSLVHNNANTYLSWYLQKPGQSPQSLIYKVSNRFSGVPDRFSGSGSGTDFTLKISRVEAEDVGVYYCGQGTQYPFTFGSGTKVEIKGGSGSSGSGGRTVAAPSVFIFPPSDEQLKSGTASVVCLLNNFYPREAKVQWKVDNALQSGNSQESVTEQDSKDSTYSLSSTLTLSKADYEKHKVYACEVTHQGLSSPVTKSFNRGECDKTHTCPPCPAPEAAGGPSVFLFPPKPKDTLMISRTPEVTCVVVDVSHEDPEVKFNWYVDGVEVHNAKTKPREEQYNSTYRVVSVLTVLHQDWLNGKEYKCKVSNKALPAPIEKTISKAKGQPREPQVYTLPPSRDELTKNQVSLTCLVKGFYPSDIAVEWESNGQPENNYKTTPPVLDSDGSFFLYSKLTVDKSRWQQGNVFSCSVMHEALHNRFTQKSLSLSPG

SEQ ID NO: 392 - protein, 226 aa, Artificial Sequence
  Fc2 of the so-called CODV-Fab-TL1 "hz20G6xhz7G3" antibody-like binding protein
DKTHTCPPCPAPEAAGGPSVFLFPPKPKDTLMISRTPEVTCVVVDVSHEDPEVKFNWYVDGVEVHNAKTKPREEQYNSTYRVVSVLTVLHQDWLNGKEYKCKVSNKALPAPIEKTISKAKGQPREPQVYTLPPSRDELTKNQVSLTCLVKGFYPSDIAVEWESNGQPENNYKTTPPVLDSDGSFFLYSKLTVDKSRWQQGNVFSCSVMHEALHNRFTQKSLSLSPG

SEQ ID NO: 393 - protein, 570 aa, Artificial Sequence
  polypeptide III of the so-called CODV-Fab-TL1 "hz20G6xhz7G3" antibody-like binding protein
QVQLVESGGGVVQPGRSLRLSCAASGFTFTKAWMHWVRQAPGKQLEWVAQIKDKSNSYATYYADSVKGRFTISRDDSKNTLYLQMNSLRAEDTAVYYCRGVYYALSPFDYWGQGTLVTVSSEVQLVQSGAEVKKPGESLKISCKGSGYSFTDYYMKWARQMPGKGLEWMGDIIPSSGATFYNQKFKGQVTISADKSISTTYLQWSSLKASDTAMYYCARSHLLRASWFAYWGQGTMVTVSSASTKGPSVFPLAPSSKSTSGGTAALGCLVKDYFPEPVTVSWNSGALTSGVHTFPAVLQSSGLYSLSSVVTVPSSSLGTQTYICNVNHKPSNTKVDKKVEPKSCDKTHTCPPCPAPEAAGGPSVFLFPPKPKDTLMISRTPEVTCVVVDVSHEDPEVKFNWYVDGVEVHNAKTKPREEQYNSTYRVVSVLTVLHQDWLNGKEYKCKVSNKALPAPIEKTISKAKGQPREPQVYTLPPSRDELTKNQVSLTCLVKGFYPSDIAVEWESNGQPENNYKTTPPVLDSDGSFFLYSKLTVDKSRWQQGNVFSCSVMHEALHNHYTQKSLSLSPG

SEQ ID NO: 394 - protein, 231 aa, Artificial Sequence
  Fc region of the so-called CODV-Fab-TL1 "hz20G6xhz7G3" antibody-like binding protein
EPKSCDKTHTCPPCPAPEAAGGPSVFLFPPKPKDTLMISRTPEVTCVVVDVSHEDPEVKFNWYVDGVEVHNAKTKPREEQYNSTYRVVSVLTVLHQDWLNGKEYKCKVSNKALPAPIEKTISKAKGQPREPQVYTLPPSRDELTKNQVSLTCLVKGFYPSDIAVEWESNGQPENNYKTTPPVLDSDGSFFLYSKLTVDKSRWQQGNVFSCSVMHEALHNHYTQKSLSLSPG

SEQ ID NO: 395 - protein, 570 aa, Artificial Sequence
  polypeptide II of the so-called CODV-Fab-OL1 "hz20G6xhz7G3" antibody-like binding protein
QVQLVESGGGVVQPGRSLRLSCAASGFTFTKAWMHWVRQAPGKQLEWVAQIKDKSNSYATYYADSVKGRFTISRDDSKNTLYLQMNSLRAEDTAVYYCRGVYYALSPFDYWGQGTLVTVSSEVQLVQSGAEVKKPGESLKISCKGSGYSFTDYYMKWARQMPGKGLEWMGDIIPSSGATFYNQKFKGQVTISADKSISTTYLQWSSLKASDTAMYYCARSHLLRASWFAYWGQGTMVTVSSASTKGPSVFPLAPSSKSTSGGTAALGCLVKDYFPEPVTVSWNSGALTSGVHTFPAVLQSSGLYSLSSVVTVPSSSLGTQTYICNVNHKPSNTKVDKKVEPKSCDKTHTCPPCPAPEAAGGPSVFLFPPKPKDTLMISRTPEVTCVVVDVSHEDPEVKFNWYVDGVEVHNAKTKPREEQYNSTYRVVSVLTVLHQDWLNGKEYKCKVSNKALPAPIEKTISKAKGQPREPQVYTLPPCRDELTKNQVSLWCLVKGFYPSDIAVEWESNGQPENNYKTTPPVLDSDGSFFLYSKLTVDKSRWQQGNVFSCSVMHEALHNRFTQKSLSLSPG

SEQ ID NO: 396 - protein, 231 aa, Artificial Sequence
  Fc region of the so-called CODV-Fab-OL1 "hz20G6xhz7G3" antibody-like binding protein
EPKSCDKTHTCPPCPAPEAAGGPSVFLFPPKPKDTLMISRTPEVTCVVVDVSHEDPEVKFNWYVDGVEVHNAKTKPREEQYNSTYRVVSVLTVLHQDWLNGKEYKCKVSNKALPAPIEKTISKAKGQPREPQVYTLPPCRDELTKNQVSLWCLVKGFYPSDIAVEWESNGQPENNYKTTPPVLDSDGSFFLYSKLTVDKSRWQQGNVFSCSVMHEALHNRFTQKSLSLSPG

SEQ ID NO: 397 - protein, 228 aa, Artificial Sequence
  Fc3 of the so-called CODV-Fab-OL1 "hz20G6xhz7G3" antibody-like binding protein
GSDKTHTCPPCPAPEAAGGPSVFLFPPKPKDTLMISRTPEVTCVVVDVSHEDPEVKFNWYVDGVEVHNAKTKPREEQYNSTYRVVSVLTVLHQDWLNGKEYKCKVSNKALPAPIEKTISKAKGQPREPQVCTLPPSRDELTKNQVSLSCAVKGFYPSDIAVEWESNGQPENNYKTTPPVLDSDGSFFLVSKLTVDKSRWQQGNVFSCSVMHEALHNHYTQKSLSLSPG

SEQ ID NO: 398 - protein, 228 aa, Artificial Sequence
  Fc3 of the so-called CODV-Fab-OL1a "hz20G6xhz7G3"
GSDKTHTCPPCPAPEAAGGPSVFLFPPKPKDTLMISRTPEVTCVVVDVSHEDPEVKFNWYVDGVEVHNAKTKPREEQYNSTYRVVSVLTVLHQDWLNGKEYKCKVSNKALPAPIEKTISKAKGQPREPQVCTLPPSRDELTKNQVSLSCAVKGFYPSDIAVEWESNGQPENNYKTTPPVLDSDGSFFLVSKLTVDKSRWQQGNVFSCSVMHEALHNRFTQKSLSLSPG

SEQ ID NO: 399 - protein, 570 aa, Artificial Sequence
  polypeptide of formula II of the so-called CODV-Fab-OL1a "hz20G6xhz7G3"
QVQLVESGGGVVQPGRSLRLSCAASGFTFTKAWMHWVRQAPGKQLEWVAQIKDKSNSYATYYADSVKGRFTISRDDSKNTLYLQMNSLRAEDTAVYYCRGVYYALSPFDYWGQGTLVTVSSEVQLVQSGAEVKKPGESLKISCKGSGYSFTDYYMKWARQMPGKGLEWMGDIIPSSGATFYNQKFKGQVTISADKSISTTYLQWSSLKASDTAMYYCARSHLLRASWFAYWGQGTMVTVSSASTKGPSVFPLAPSSKSTSGGTAALGCLVKDYFPEPVTVSWNSGALTSGVHTFPAVLQSSGLYSLSSVVTVPSSSLGTQTYICNVNHKPSNTKVDKKVEPKSCDKTHTCPPCPAPEAAGGPSVFLFPPKPKDTLMISRTPEVTCVVVDVSHEDPEVKFNWYVDGVEVHNAKTKPREEQYNSTYRVVSVLTVLHQDWLNGKEYKCKVSNKALPAPIEKTISKAKGQPREPQVYTLPPCRDELTKNQVSLWCLVKGFYPSDIAVEWESNGQPENNYKTTPPVLDSDGSFFLYSKLTVDKSRWQQGNVFSCSVMHEALHNHYTQKSLSLSPG

SEQ ID NO: 400 - protein, 231 aa, Artificial Sequence
  Fc3 of the so-called CODV-Fab-OL1a "hz20G6xhz7G3" antibody-like binding protein
EPKSCDKTHTCPPCPAPEAAGGPSVFLFPPKPKDTLMISRTPEVTCVVVDVSHEDPEVKFNWYVDGVEVHNAKTKPREEQYNSTYRVVSVLTVLHQDWLNGKEYKCKVSNKALPAPIEKTISKAKGQPREPQVYTLPPCRDELTKNQVSLWCLVKGFYPSDIAVEWESNGQPENNYKTTPPVLDSDGSFFLYSKLTVDKSRWQQGNVFSCSVMHEALHNHYTQKSLSLSPG